European Patent Application EP 4 219 521 A2, published August 2, 2023. Title: Cellular growth and proliferation promoting peptides, and uses thereof. Applicant: NURITAS LIMITED. Application WO PCT/EP2016/067097, filed July 18, 2016. The sequence listing filed with the application follows.

SEQUENCE LISTING (775 sequences)

SEQ ID NO: 1 - protein, 459 aa, Pisum sativum
MAATTMKASFPLLMLMGISFLASVCVSSRSDPQNPFIFKSNKFQTLFENENGHIRLLQKFDQRSKIFENLQNYRLLEYKSKPHTIFLPQHTDADYILVVLSGKAILTVLKPDDRNSFNLERGDTIKLPAGTIAYLVNRDDNEELRVLDLAIPVNRPGQLQSFLLSGNQNQQNYLSGFSKNILEASFNTDYEEIEKVLLEEHEKETQHRRSLKDKRQQSQEENVIVKLSRGQIEELSKNAKSTSKKSVSSESEPFNLRSRGPIYSNEFGKFFEITPEKNPQLQDLDIFVNSVEIKEGSLLLPHYNSRAIVIVTVNEGKGDFELVGQRNENQQEQRKEDDEEEEQGEEEINKQVQNYKAKLSSGDVFVIPAGHPVAVKASSNLDLLGFGINAENNQRNFLAGDEDNVISQIQRPVKELAFPGSAQEVDRILENQKQSHFADAQPQQRERGSRETRDRLSSV

SEQ ID NO: 2 - protein, 613 aa, Pisum sativum
MATTIKSRFPLLLLLGIIFLASVVCVTYANYDEGSEPRVPAQRERGRQEGEKEEKRHGEWRPSYEKEEDEEEGQRERGRQEGEKEEKRHGEWRPSYEKQEDEEEKQKYRYQREKEDEEEKQKYQYQREKKEQKEVQPGRERWEREEDEEQVDEEWRGSQRREDPEERARLRHREERTKRDRRHQREGEEEERSSESQERRNPFLFKSNKFLTLFENENGHIRLLQRFDKRSDLFENLQNYRLVEYRAKPHTIFLPQHIDADLILVVLSGKAILTVLSPNDRNSYNLERGDTIKLPAGTTSYLVNQDDEEDLRLVDLVIPVNGPGKFEAFDLAKNKNQYLRGFSKNILEASYNTRYETIEKVLLEEQEKDRKRRQQGEETDAIVKVSREQIEELKKLAKSSSKKSLPSEFEPINLRSHKPEYSNKFGKLFEITPEKKYPQLQDLDLFVSCVEINEGALMLPHYNSRAIVVLLVNEGKGNLELLGLKNEQQEREDRKERNNEVQRYEARLSPGDVVIIPAGHPVAITASSNLNLLGFGINAENNERNFLSGSDDNVISQIENPVKELTFPGSVQEINRLIKNQKQSHFANAEPEQKEQGSQGKRSPLSSILGTFY

SEQ ID NO: 3 - protein, 609 aa, Oryza sativa
MSALTTSQLATSATGFGIADRSAPSSLLRHGFQGLKPRSPAGGDATSLSVTTSARATPKQQRSVQRGSRRFPSVVVYATGAGMNVVFVGAEMAPWSKTGGLGDVLGGLPPAMAANGHRVMVISPRYDQYKDAWDTSVVAEIKVADRYERVRFFHCYKRGVDRVFIDHPSFLEKVWGKTGEKIYGPDTGVDYKDNQMRFSLLCQAALEAPRILNLNNNPYFKGTYGEDVVFVCNDWHTGPLASYLKNNYQPNGIYRNAKVAFCIHNISYQGRFAFEDYPELNLSERFRSSFDFIDGYDTPVEGRKINWMKAGILEADRVLTVSPYYAEELISGIARGCELDNIMRLTGITGIVNGMDVSEWDPSKDKYITAKYDATTAIEAKALNKEALQAEAGLPVDRKIPLIAFIGRLEEQKGPDVMAAAIPELMQEDVQIVLLGTGKKKFEKLLKSMEEKYPGKVRAVVKFNAPLAHLIMAGADVLAVPSRFEPCGLIQLQGMRYGTPCACASTGGLVDTVIEGKTGFHMGRLSVDCKVVEPSDVKKVAATLKRAIKVVGTPAYEEMVRNCMNQDLSWKGPAKNWENVLLGLGVAGSAPGIEGDEIAPLAKENVAAP

SEQ ID NO: 4 - protein, 499 aa, Oryza sativa
MASSVFSRFSIYFCVLLLCHGSMAQLFNPSTNPWHSPRQGSFRECRFDRLQAFEPLRKVRSEAGVTEYFDEKNELFQCTGTFVIRRVIQPQGLLVPRYTNIPGVVYIIQGRGSMGLTFPGCPATYQQQFQQFSSQGQSQSQKFRDEHQKIHQFRQGDIVALPAGVAHWFYNDGDAPIVAVYVYDVNNNANQLEPRQKEFLLAGNNNRAQQQQVYGSSIEQHSGQNIFSGFGVEMLSEALGINAVAAKRLQSQNDQRGEIIHVKNGLQLLKPTLTQQQEQAQAQDQYQQVQYSERQQTSSRWNGLEENFCTIKVRVNIENPSRADSYNPRAGRITSVNSQKFPILNLIQMSATRVNLYQNAILSPFWNVNAHSLVYMIQGRSRVQVVSNFGKTVFDGVLRPGQLLIIPQHYAVLKKAEREGCQYIAIKTNANAFVSHLAGKNSVFRALPVDVVANAYRISREQARSLKNNRGEEHGAFTPRFQQQYYPGLSNESESETSE

SEQ ID NO: 5 - protein, 186 aa, Oryza sativa
MASKVVFFAAALMAAMVAISGAQLSESEMRFRDRQCQREVQDSPLDACRQVLDRQLTGRERFQPMFRRPGALGLRMQCCQQLQDVSRECRCAAIRRMVRSYEESMPMPLEQGWSSSSSEYYGGEGSSSEQGYYGEGSSEEGYYGEQQQQPGMTRVRLTRARQYAAQLPSMCRVEPQQCSIFAAGQY

SEQ ID NO: 6 - protein, 500 aa, Oryza sativa
MATIAFSRLSIYFCVLLLCHGSMAQLFGPNVNPWHNPRQGGFRECRFDRLQAFEPLRRVRSEAGVTEYFDEKNEQFQCTGTFVIRRVIEPQGLLVPRYSNTPGMVYIIQGRGSMGLTFPGCPATYQQQFQQFLPEGQSQSQKFRDEHQKIHQFRQGDIVALPAGVAHWFYNEGDAPVVALYVFDLNNNANQLEPRQKEFLLAGNNNREQQMYGRSIEQHSGQNIFSGFNNELLSEALGVNALVAKRLQGQNDQRGEIIRVKNGLKLLRPAFAQQQEQAQQQEQAQAQYQVQYSEEQQPSTRCNGLDENFCTIKARLNIENPSHADTYNPRAGRITRLNSQKFPILNLVQLSATRVNLYQNAILSPFWNVNAHSLVYIVQGHARVQVVSNLGKTVFNGVLRPGQLLIIPQHYVVLKKAEHEGCQYISFKTNANSMVSHLAGKNSIFRAMPVDVIANAYRISREQARSLKNNRGEELGAFTPRYQQQTYPGFSNESENEALE

SEQ ID NO: 7 - protein, 861 aa, Pisum sativum
MFSGVTGILNRGHKIKGTVVLMRKNVLDINSLTTVGGVIGQGFDILGSTVDNLTAFLGRSVSLQLISATKPDATGKGKLGKATFLEGIISSLPTLGAGQSAFKIHFEWDDDMGIPGAFYIKNFMQTEFFLVSLTLDDIPNHGSIYFVCNSWIYNAKHHKIDRIFFANQTYLPSETPAPLVHYREEELNNLRGDGTGERKEWERIYDYDVYNDLGNPDSGENHARPVLGGSETYPYPRRGRTGRKPTRKDPNSESRSDYVYLPRDEAFGHLKSSDFLTYGLKAVSQNVVPALESVFFDLNFTPNEFDSFDEVHGLYEGGIKLPTNILSQISPLPVLKEIFRTDGENTLKYPPPKVIQVSRSGWMTDEEFAREMLAGVNPNVICCLQEFPPRSKLDSQIYGDHTSKISKEHLEPNLEGLTVEEAIQNKKLFLLDHHDSIMPYLRRINSTSTKAYATRTILFLNNNQNLKPLAIELSLPHPQGDEHGAVSYVYQPALEGVESSIWLLAKAYVIVNDSCYHQLVSHWLNTHAVVEPFVIATNRHLSCLHPIYKLLYPHYRDTMNINSLARLSLVNDGGIIEKTFLWGRYSMEMSSKVYKNWVFTEQALPADLIKRGMAIEDPSSPCGVKLVVEDYPYAVDGLEIWAIIKTWVQDYVSLYYTSDEKLRQDSELQAWWKELVEVGHGDKKNEPWWPKMQTREDLIEVCSIVIWTASALHAAVNFGQYSYGGLILNRPTLSRRFMPEKGSAEFEELVKSPQKAYLKTITPKFQTLIDLSVIEILSRHASDELYLGERDNPNWTSDKRALEAFKKFGNKLAEIEKKLTQRNNDEKLRNRHGPVEMPYTLLYPSSKEGLTFRGIPNSISI

SEQ ID NO: 8 - protein, 517 aa, Pisum sativum
MAKLLALSLSFCFLLLGGCFALREQPQQNECQLERLDALEPDNRIESEGGLIETWNPNNKQFRCAGVALSRATLQRNALRRPYYSNAPQEIFIQQGNGYFGMVFPGCPETFEEPQESEQGEGRRYRDRHQKVNRFREGDIIAVPTGIVFWMYNDQDTPVIAVSLTDIRSSNNQLDQMPRRFYLAGNHEQEFLQYQHQQGGKQEQENEGNNIFSGFKRDYLEDAFNVNRHIVDRLQGRNEDEEKGAIVKVKGGLSIISPPEKQARHQRGSRQEEDEDEEKQPRHQRGSRQEEEEDEDEERQPRHQRRRGEEEEEDKKERGGSQKGKSRRQGDNGLEETVCTAKLRLNIGPSSSPDIYNPEAGRIKTVTSLDLPVLRWLKLSAEHGSLHKNAMFVPHYNLNANSIIYALKGRARLQVVNCNGNTVFDGELEAGRALTVPQNYAVAAKSLSDRFSYVAFKTNDRAGIARLAGTSSVINNLPLDVVAATFNLQRNEARQLKSNNPFKFLVPARESENRASA

SEQ ID NO: 9 - protein, 275 aa, Pisum sativum
DNAEIEKILLEEHEKETHHRRGLRDKRQQSQEKNVIVKVSKKQIEELSKNAKSSSKKSVSSRSEPFNLKSSDPIYSNQYGKFFEITPKKNPQLQDLDIFVNYVEIKEGSLWLPHYNSRAIVIVTVNEGKGDFELVGQRNENQQGLREEDDEEEEQREEETKNQVQSYKAKLTPGDVFVIPAGHPVAVRASSNLNLLGFGINAENNQRNFLAGEEDNVISQIQKQVKDLTFPGSAQEVDRLLENQKQSYFANAQPQQRETRSQEIKEHLYSILGAF

SEQ ID NO: 10 - protein, 438 aa, Pisum sativum
MAATPIKPLMLLAIAFLASVCVSSRSDQENPFIFKSNRFQTLYENENGHIRLLQKFDKRSKIFENLQNYRLLEYKSKPRTLFLPQYTDADFILVVLSGKATLTVLKSNDRNSFNLERGDTIKLPAGTIAYLANRDDNEDLRVLDLTIPVNKPGQLQSFLLSGTQNQPSLLSGFSKNILEAAFNTNYEEIEKVLLEQQEQEPQHRRSLKDRRQEINEENVIVKVSREQIEELSKNAKSSSKKSVSSESGPFNLRSRNPIYSNKFGKFFEITPEKNQQLQDLDIFVNSVDIKEGSLLLPNYNSRAIVIVTVTEGKGDFELVGQRNENQGKENDKEEEQEEETSKQVQLYRAKLSPGDVFVIPAGHPVAINASSDLNLIGFGINAENNERNFLAGEEDNVISQVERPVKELAFPGSSHEVDRLLKNQKQSYFANAQPLQRE

SEQ ID NO: 11 - protein, 499 aa, Oryza sativa
MASINRPIVFFTVCLFLLCNGSLAQQLLGQSTSQWQSSRRGSPRECRFDRLQAFEPIRSVRSQAGTTEFFDVSNEQFQCTGVSVVRRVIEPRGLLLPHYTNGASLVYIIQGRGITGPTFPGCPESYQQQFQQSGQAQLTESQSQSQKFKDEHQKIHRFRQGDVIALPAGVAHWCYNDGEVPVVAIYVTDLNNGANQLDPRQRDFLLAGNKRNPQAYRREVEERSQNIFSGFSTELLSEALGVSSQVARQLQCQNDQRGEIVRVEHGLSLLQPYASLQEQEQGQVQSRERYQEGQYQQSQYGSGCSNGLDETFCTLRVRQNIDNPNRADTYNPRAGRVTNLNTQNFPILSLVQMSAVKVNLYQNALLSPFWNINAHSVVYITQGRARVQVVNNNGKTVFNGELRRGQLLIIPQHYAVVKKAQREGCAYIAFKTNPNSMVSHIAGKSSIFRALPNDVLANAYRISREEAQRLKHNRGDEFGAFTPIQYKSYQDVYNAAESS

SEQ ID NO: 12 - protein, 499 aa, Oryza sativa
MASINRPIVFFTVCLFLLCDGSLAQQLLGQSTSQWQSSRRGSPRGCRFDRLQAFEPIRSVRSQAGTTEFFDVSNELFQCTGVSVVRRVIEPRGLLLPHYTNGASLVYIIQGRGITGPTFPGCPETYQQQFQQSGQAQLTESQSQSHKFKDEHQKIHRFRQGDVIALPAGVAHWCYNDGEVPVVAIYVTDINNGANQLDPRQRDFLLAGNKRNPQAYRREVEEWSQNIFSGFSTELLSEAFGISNQVARQLQCQNDQRGEIVRVERGLSLLQPYASLQEQEQGQMQSREHYQEGGYQQSQYGSGCPNGLDETFCTMRVRQNIDNPNRADTYNPRAGRVTNLNSQNFPILNLVQMSAVKVNLYQNALLSPFWNINAHSIVYITQGRAQVQVVNNNGKTVFNGELRRGQLLIVPQHYVVVKKAQREGCAYIAFKTNPNSMVSHIAGKSSIFRALPTDVLANAYRISREEAQRLKHNRGDEFGAFTPLQYKSYQDVYNVAESS

SEQ ID NO: 13 - protein, 160 aa, Oryza sativa
MASNKVVFSVLLLAVVSVLAATATMAEYHHQDQVVYTPGPLCQPGMGYPMYPLPRCRALVKRQCVGRGTAAAAEQVRRDCCRQLAAVDDSWCRCEAISHMLGGIYRELGAPDVGHPMSEVFRGCRRGDLERAAASLPAFCNVDIPNGGGGVCYWLARSGY

SEQ ID NO: 14 - protein, 336 aa, Staphylococcus aureus
MKGKFLKVSSLFVATLTTATLVSSPAANALSSKAMDNHPQQTQSSKQQTPKIQKGGNLKPLEQREHANVILPNNDRHQITDTTNGHYAPVTYIQVEAPTGTFIASGVVVGKDTLLTNKHVVDATHGDPHALKAFPSAINQDNYPNGGFTAEQITKYSGEGDLAIVKFSPNEQNKHIGEVVKPATMSNNAETQVNQNITVTGYPGDKPVATMWESKGKITYLKGEAMQYDLSTTGGNSGSPVFNEKNEVIGIHWGGVPNEFNGAVFINENVRNFLKQNIEDIHFANDDQPNNPDNPDNPNNPDNPNNPDEPNNPDNPNNPDNPDNGDNNNSDNPDAA

SEQ ID NO: 15 - protein, 13 aa, synthetic construct
  REGION 1..13: note = FRAGMENT OF SEQ ID 1
QNYLSGFSKNILE

SEQ ID NO: 16 - protein, 20 aa, synthetic construct
  REGION 1..20: note = FRAGMENT OF SEQ ID 1
TIKLPAGTIAYLVNRDDNEE

SEQ ID NO: 17 - protein, 15 aa, synthetic construct
  REGION 1..15: note = FRAGMENT OF SEQ ID 1
LAIPVNRPGQLQSFL

SEQ ID NO: 18 - protein, 11 aa, synthetic construct
  REGION 1..11: note = FRAGMENT OF SEQ ID 1
AIPVNRPGQLQ

SEQ ID NO: 19 - protein, 9 aa, synthetic construct
  REGION 1..9: note = FRAGMENT OF SEQ ID 1
PAGHPVAVK

SEQ ID NO: 20 - protein, 19 aa, synthetic construct
  REGION 1..19: note = FRAGMENT FOR SEQ ID 1
VQNYKAKLSSGDVFVIPAG

SEQ ID NO: 21 - protein, 24 aa, synthetic construct
  REGION 1..24: note = FRAGMENT OF SEQ ID 1
NNQRNFLAGDEDNVISQIQRPVKE

SEQ ID NO: 22 - protein, 23 aa, synthetic construct
  REGION 1..23: note = FRAGMENT OF SEQ ID 1
INKQVQNYKAKLSSGDVFVIPAG

SEQ ID NO: 23 - protein, 10 aa, synthetic construct
  REGION 1..10: note = FRAGMENT OF SEQ ID 1
LAIPVNRPGQ

SEQ ID NO: 24 - protein, 20 aa, synthetic construct
  REGION 1..20: note = FRAGMENT OF SEQ ID 1
NFLAGDEDNVISQIQRPVKE

SEQ ID NO: 25 - protein, 15 aa, synthetic construct
  REGION 1..15: note = FRAGMENT OF SEQ ID 1
DLAIPVNRPGQLQSF

SEQ ID NO: 26 - protein, 11 aa, synthetic construct
  REGION 1..11: note = FRAGMENT OF SEQ ID 1
VIPAGHPVAVK

SEQ ID NO: 27 - protein, 21 aa, synthetic construct
  REGION 1..21: note = FRAGMENT OF SEQ ID 1
DTIKLPAGTIAYLVNRDDNEE

SEQ ID NO: 28 - protein, 14 aa, synthetic construct
  REGION 1..14: note = FRAGMENT OF SEQ ID 1
LAIPVNRPGQLQSF

SEQ ID NO: 29 - protein, 21 aa, synthetic construct
  REGION 1..21: note = FRAGMENT OF SEQ ID 1
KQVQNYKAKLSSGDVFVIPAG

SEQ ID NO: 30 - protein, 23 aa, synthetic construct
  REGION 1..23: note = FRAGMENT SEQ ID 1
RGDTIKLPAGTIAYLVNRDDNEE

SEQ ID NO: 31 - protein, 19 aa, synthetic construct
  REGION 1..19: note = FRAGMENT OF SEQ ID 1
FLAGDEDNVISQIQRPVKE

SEQ ID NO: 32 - protein, 13 aa, synthetic construct
  REGION 1..13: note = FRAGMENT OF SEQ ID 1
LAIPVNRPGQLQS

SEQ ID NO: 33 - protein, 15 aa, synthetic construct
  REGION 1..15: note = FRAGMENT OF SEQ ID 1
VLDLAIPVNRPGQLQ

SEQ ID NO: 34 - protein, 13 aa, synthetic construct
  REGION 1..13: note = FRAGMENT OF SEQ ID 1
DLAIPVNRPGQLQ

SEQ ID NO: 35 - protein, 13 aa, synthetic construct
  REGION 1..13: note = FRAGMENT OF SEQ ID 1
VFVIPAGHPVAVK

SEQ ID NO: 36 - protein, 20 aa, synthetic construct
  REGION 1..20: note = FRAGMENT OF SEQ ID 1
TIFLPQHTDADYILVVLSGK

SEQ ID NO: 37 - protein, 23 aa, synthetic construct
  REGION 1..23: note = FRAGMENT OF SEQ ID 1
NQRNFLAGDEDNVISQIQRPVKE

SEQ ID NO: 38 - protein, 12 aa, synthetic construct
  REGION 1..12: note = FRAGMENT OF SEQ ID 1
LAIPVNRPGQLQ

SEQ ID NO: 39 - protein, 17 aa, synthetic construct
  REGION 1..17: note = FRAGMENT OF SEQ ID 1
HPVAVKASSNLDLLGFG

SEQ ID NO: 40 - protein, 11 aa, synthetic construct
  REGION 1..11: note = FRAGMENT OF SEQ ID 1
LAIPVNRPGQL

SEQ ID NO: 41 - protein, 12 aa, synthetic construct
  REGION 1..12: note = FRAGMENT SEQ ID 1
DLAIPVNRPGQL

SEQ ID NO: 42 - protein, 24 aa, synthetic construct
  REGION 1..24: note = FRAGMENT OF SEQ ID 1
SKPHTIFLPQHTDADYILVVLSGK

SEQ ID NO: 43 - protein, 12 aa, synthetic construct
  REGION 1..12: note = FRAGMENT OF SEQ ID 1
FVIPAGHPVAVK

SEQ ID NO: 44 - protein, 14 aa, synthetic construct
  REGION 1..14: note = FRAGMENT OF SEQ ID 1
DLAIPVNRPGQLQS

SEQ ID NO: 45 - protein, 22 aa, synthetic construct
  REGION 1..22: note = FRAGMENT OF SEQ ID 1
SGDVFVIPAGHPVAVKASSNLD

SEQ ID NO: 46 - protein, 13 aa, synthetic construct
  REGION 1..13: note = FRAGMENT OF SEQ ID 1
AIPVNRPGQLQSF

SEQ ID NO: 47 - protein, 13 aa, synthetic construct
  REGION 1..13: note = FRAGMENT OF SEQ ID 1
ELAFPGSAQEVDR

SEQ ID NO: 48 - protein, 18 aa, synthetic construct
  REGION 1..18: note = FRAGMENT OF SEQ ID 1
LAIPVNRPGQLQSFLLSG

SEQ ID NO: 49 - protein, 24 aa, synthetic construct
  REGION 1..24: note = FRAGMENT OF SEQ ID 1
VFVIPAGHPVAVKASSNLDLLGFG

SEQ ID NO: 50 - protein, 8 aa, synthetic construct
  REGION 1..8: note = FRAGMENT OF SEQ ID 1
AGHPVAVK

SEQ ID NO: 51 - protein, 21 aa, synthetic construct
  REGION 1..21: note = FRAGMENT OF SEQ ID 1
HPVAVKASSNLDLLGFGINAE

SEQ ID NO: 52 - protein, 22 aa, synthetic construct
  REGION 1..22: note = FRAGMENT SEQ ID 1
LAIPVNRPGQLQSFLLSGNQNQ

SEQ ID NO: 53 - protein, 10 aa, synthetic construct
  REGION 1..10: note = FRAGMENT SEQ ID 1
SGDVFVIPAG

SEQ ID NO: 54 - protein, 20 aa, synthetic construct
  REGION 1..20: note = FRAGMENT OF SEQ ID 1
GSLLLPHYNSRAIVIVTVNE

SEQ ID NO: 55 - protein, 19 aa, synthetic construct
  REGION 1..19: note = FRAGMENT OF SEQ ID 1
NFLAGDEDNVISQIQRPVK

SEQ ID NO: 56 - protein, 14 aa, synthetic construct
  REGION 1..14: note = FRAGMENT SEQ ID 1
SGDVFVIPAGHPVA

SEQ ID NO: 57 - protein, 16 aa, synthetic construct
  REGION 1..16: note = FRAGMENT SEQ ID 1
GSLLLPHYNSRAIVIV

SEQ ID NO: 58 - protein, 20 aa, synthetic construct
  REGION 1..20: note = FRAGMENT SEQ ID 1
RGDTIKLPAGTIAYLVNRDD

SEQ ID NO: 59 - protein, 16 aa, synthetic construct
  REGION 1..16: note = FRAGMENT OF SEQ ID 1
SGDVFVIPAGHPVAVK

SEQ ID NO: 60 - protein, 18 aa, synthetic construct
  REGION 1..18: note = FRAGMENT SEQ ID 1
LSSGDVFVIPAGHPVAVK

SEQ ID NO: 61 - protein, 13 aa, synthetic construct
  REGION 1..13: note = FRAGMENT OF SEQ ID 1
LDLAIPVNRPGQL

SEQ ID NO: 62 - protein, 10 aa, synthetic construct
  REGION 1..10: note = FRAGMENT OF SEQ ID 1
AIPVNRPGQL

SEQ ID NO: 63 - protein, 16 aa, synthetic construct
  REGION 1..16: note = FRAGMENT OF SEQ ID 1
LAIPVNRPGQLQSFLL

SEQ ID NO: 64 - protein, 22 aa, synthetic construct
  REGION 1..22: note = FRAGMENT OF SEQ ID 1
PHTIFLPQHTDADYILVVLSGK

SEQ ID NO: 65 - protein, 19 aa, synthetic construct
  REGION 1..19: note = FRAGMENT OF SEQ ID 1
VFVIPAGHPVAVKASSNLD

SEQ ID NO: 66 - protein, 17 aa, synthetic construct
  REGION 1..17: note = FRAGMENT OF SEQ ID 1
LAIPVNRPGQLQSFLLS

SEQ ID NO: 67 - protein, 17 aa, synthetic construct
  REGION 1..17: note = FRAGMENT OF SEQ ID 1
VLDLAIPVNRPGQLQSF

SEQ ID NO: 68 - protein, 12 aa, synthetic construct
  REGION 1..12: note = FRAGMENT OF SEQ ID 1
AIPVNRPGQLQS

SEQ ID NO: 69 - protein, 20 aa, synthetic construct
  REGION 1..20: note = FRAGMENT OF SEQ ID 1
DTIKLPAGTIAYLVNRDDNE

SEQ ID NO: 70 - protein, 17 aa, synthetic construct
  REGION 1..17: note = FRAGMENT OF SEQ ID 1
NYKAKLSSGDVFVIPAG

SEQ ID NO: 71 - protein, 19 aa, synthetic construct
  REGION 1..19: note = FRAGMENT OF SEQ ID 1
GKAILTVLKPDDRNSFNLE

SEQ ID NO: 72 - protein, 17 aa, synthetic construct
  REGION 1..17: note = FRAGMENT OF SEQ ID 1
YKSKPHTIFLPQHTDAD

SEQ ID NO: 73 - protein, 11 aa, synthetic construct
  REGION 1..11: note = FRAGMENT OF SEQ ID 1
ASSNLDLLGFG

SEQ ID NO: 74 - protein, 13 aa, synthetic construct
  REGION 1..13: note = FRAGMENT OF SEQ ID 1
DEEEEQGEEEINK

SEQ ID NO: 75 - protein, 15 aa, synthetic construct
  REGION 1..15: note = FRAGMENT OF SEQ ID 1
YKSKPHTIFLPQHTD

SEQ ID NO: 76 - protein, 10 aa, synthetic construct
  REGION 1..10: note = FRAGMENT OF SEQ ID 1
VLDLAIPVNR

SEQ ID NO: 77 - protein, 25 aa, synthetic construct
  REGION 1..25: note = FRAGMENT OF SEQ ID 1
FFEITPEKNPQLQDLDIFVNSVEIK

SEQ ID NO: 78 - protein, 14 aa, synthetic construct
  REGION 1..14: note = FRAGMENT OF SEQ ID 1
TIFLPQHTDADYIL

SEQ ID NO: 79 - protein, 16 aa, synthetic construct
  REGION 1..16: note = FRAGMENT OF SEQ ID 1
SFLLSGNQNQQNYLSG

SEQ ID NO: 80 - protein, 18 aa, synthetic construct
  REGION 1..18: note = FRAGMENT OF SEQ ID 1
SFLLSGNQNQQNYLSGFS

SEQ ID NO: 81 - protein, 19 aa, synthetic construct
  REGION 1..19: note = FRAGMENT OF SEQ ID 1
NQQEQRKEDDEEEEQGEEE

SEQ ID NO: 82 - protein, 10 aa, synthetic construct
  REGION 1..10: note = FRAGMENT OF SEQ ID 1
EEQGEEEINK

SEQ ID NO: 83 - protein, 9 aa, synthetic construct
  REGION 1..9: note = FRAGMENT OF SEQ ID 1
SRGPIYSNE

SEQ ID NO: 84 - protein, 15 aa, synthetic construct
  REGION 1..15: note = FRAGMENT OF SEQ ID 1
EDDEEEEQGEEEINK

SEQ ID NO: 85 - protein, 14 aa, synthetic construct
  REGION 1..14: note = FRAGMENT OF SEQ ID 1
DDEEEEQGEEEINK

SEQ ID NO: 86 - protein, 15 aa, synthetic construct
  REGION 1..15: note = FRAGMENT OF SEQ ID 1
KEDDEEEEQGEEEIN

SEQ ID NO: 87 - protein, 12 aa, synthetic construct
  REGION 1..12: note = FRAGMENT OF SEQ ID 1
KEDDEEEEQGEE

SEQ ID NO: 88 - protein, 15 aa, synthetic construct
  REGION 1..15: note = FRAGMENT OF SEQ ID 1
QRKEDDEEEEQGEEE

SEQ ID NO: 89 - protein, 16 aa, synthetic construct
  REGION 1..16: note = FRAGMENT OF SEQ ID 1
KEDDEEEEQGEEEINK

SEQ ID NO: 90 - protein, 13 aa, synthetic construct
  REGION 1..13: note = FRAGMENT OF SEQ ID 1
KEDDEEEEQGEEE

SEQ ID NO: 91 - protein, 15 aa, synthetic construct
  REGION 1..15: note = FRAGMENT OF SEQ ID 2
HPVAITASSNLNLLG

SEQ ID NO: 92 - protein, 11 aa, synthetic construct
  REGION 1..11: note = FRAGMENT OF SEQ ID 2
ASSNLNLLGFG

SEQ ID NO: 93 - protein, 13 aa, synthetic construct
  REGION 1..13: note = FRAGMENT OF SEQ ID 2
ITASSNLNLLGFG

SEQ ID NO: 94 - protein, 17 aa, synthetic construct
  REGION 1..17: note = FRAGMENT OF SEQ ID 2
ITASSNLNLLGFGINAE

SEQ ID NO: 95 - protein, 10 aa, synthetic construct
  REGION 1..10: note = FRAGMENT OF SEQ ID 2
SSNLNLLGFG

SEQ ID NO: 96 - protein, 13 aa, synthetic construct
  REGION 1..13: note = FRAGMENT OF SEQ ID 2
VDLVIPVNGPGKF

SEQ ID NO: 97 - protein, 12 aa, synthetic construct
  REGION 1..12: note = FRAGMENT OF SEQ ID 2
LVIPVNGPGKFE

SEQ ID NO: 98 - protein, 13 aa, synthetic construct
  REGION 1..13: note = FRAGMENT OF SEQ ID 2
LVIPVNGPGKFEA

SEQ ID NO: 99 - protein, 17 aa, synthetic construct
  REGION 1..17: note = FRAGMENT OF SEQ ID 2
LRLVDLVIPVNGPGKFE

SEQ ID NO: 100 - protein, 17 aa, synthetic construct
  REGION 1..17: note = FRAGMENT OF SEQ ID 2
YRAKPHTIFLPQHIDAD

SEQ ID NO: 101 - protein, 21 aa, synthetic construct
  REGION 1..21: note = FRAGMENT OF SEQ ID 2
HPVAITASSNLNLLGFGINAE

SEQ ID NO: 102 - protein, 9 aa, synthetic construct
  REGION 1..9: note = FRAGMENT OF SEQ ID 2
SNLNLLGFG

SEQ ID NO: 103 - protein, 24 aa, synthetic construct
  REGION 1..24: note = FRAGMENT OF SEQ ID 2
HPVAITASSNLNLLGFGINAENNE

SEQ ID NO: 104 - protein, 15 aa, synthetic construct
  REGION 1..15: note = FRAGMENT OF SEQ ID 2
LVDLVIPVNGPGKFE

SEQ ID NO: 105 - protein, 11 aa, synthetic construct
  REGION 1..11: note = FRAGMENT OF SEQ ID 2
LVIPVNGPGKF

SEQ ID NO: 106 - protein, 18 aa, synthetic construct
  REGION 1..18: note = FRAGMENT OF SEQ ID 2
TIKLPAGTTSYLVNQDDE

SEQ ID NO: 107 - protein, 18 aa, synthetic construct
  REGION 1..18: note = FRAGMENT OF SEQ ID 2
DLRLVDLVIPVNGPGKFE

SEQ ID NO: 108 - protein, 19 aa, synthetic construct
  REGION 1..19: note = FRAGMENT OF SEQ ID 2
EDLRLVDLVIPVNGPGKFE

SEQ ID NO: 109 - protein, 17 aa, synthetic construct
  REGION 1..17: note = FRAGMENT OF SEQ ID 2
HPVAITASSNLNLLGFG

SEQ ID NO: 110 - protein, 21 aa, synthetic construct
  REGION 1..21: note = FRAGMENT OF SEQ ID 2
LVDLVIPVNGPGKFEAFDLAK

SEQ ID NO: 111 - protein, 13 aa, synthetic construct
  REGION 1..13: note = FRAGMENT OF SEQ ID 2
DNVISQIENPVKE

SEQ ID NO: 112 - protein, 24 aa, synthetic construct
  REGION 1..24: note = FRAGMENT OF SEQ ID 2
VVIIPAGHPVAITASSNLNLLGFG

SEQ ID NO: 113 - protein, 17 aa, synthetic construct
  REGION 1..17: note = FRAGMENT OF SEQ ID 2
LVDLVIPVNGPGKFEAF

SEQ ID NO: 114 - protein, 9 aa, synthetic construct
  REGION 1..9: note = FRAGMENT OF SEQ ID 2
YPQLQDLDL

SEQ ID NO: 115 - protein, 10 aa, synthetic construct
  REGION 1..10: note = FRAGMENT OF SEQ ID 2
VIPVNGPGKF

SEQ ID NO: 116 - protein, 8 aa, synthetic construct
  REGION 1..8: note = FRAGMENT OF SEQ ID 2
SKKSLPSE

SEQ ID NO: 117 - protein, 17 aa, synthetic construct
  REGION 1..17: note = FRAGMENT OF SEQ ID 2
LPQHIDADLILVVLSGK

SEQ ID NO: 118 - protein, 19 aa, synthetic construct
  REGION 1..19: note = FRAGMENT OF SEQ ID 2
RGDTIKLPAGTTSYLVNQD

SEQ ID NO: 119 - protein, 9 aa, synthetic construct
  REGION 1..9: note = FRAGMENT OF SEQ ID 2
IPVNGPGKF

SEQ ID NO: 120 - protein, 9 aa, synthetic construct
  REGION 1..9: note = FRAGMENT OF SEQ ID 2
LPQHIDADL

SEQ ID NO: 121 - protein, 10 aa, synthetic construct
  REGION 1..10: note = FRAGMENT OF SEQ ID 2
LVIPVNGPGK

SEQ ID NO: 122 - protein, 10 aa, synthetic construct
  REGION 1..10: note = FRAGMENT OF SEQ ID 2
IFLPQHIDAD

SEQ ID NO: 123 - protein, 8 aa, synthetic construct
  REGION 1..8: note = FRAGMENT OF SEQ ID 2
LPQHIDAD

SEQ ID NO: 124 - protein, 9 aa, synthetic construct
  REGION 1..9: note = FRAGMENT OF SEQ ID 2
VIPVNGPGK

SEQ ID NO: 125 - protein, 9 aa, synthetic construct
  REGION 1..9: note = FRAGMENT OF SEQ ID 2
IFLPQHIDA

SEQ ID NO: 126 - protein, 19 aa, synthetic construct
  REGION 1..19: note = FRAGMENT OF SEQ ID 2
TIKLPAGTTSYLVNQDDEE

SEQ ID NO: 127 - protein, 21 aa, synthetic construct
  REGION 1..21: note = FRAGMENT OF SEQ ID 2
HGEWRPSYEKEEDEEEGQRER

SEQ ID NO: 128 - protein, 23 aa, synthetic construct
  REGION 1..23: note = FRAGMENT OF SEQ ID 2
EKRHGEWRPSYEKEEDEEEGQRE

SEQ ID NO: 129 - protein, 19 aa, synthetic construct
  REGION 1..19: note = EKRHGEWRPSYEKEEDEEEGQRE
LPAGTTSYLVNQDDEEDLR

SEQ ID NO: 130 - protein, 16 aa, synthetic construct
  REGION 1..16: note = EKRHGEWRPSYEKEEDEEEGQRE
PSYEKEEDEEEGQRER

SEQ ID NO: 131 - protein, 12 aa, synthetic construct
  REGION 1..12: note = EKRHGEWRPSYEKEEDEEEGQRE
EKRHGEWRPSYE

SEQ ID NO: 132 - protein, 20 aa, synthetic construct
  REGION 1..20: note = EKRHGEWRPSYEKEEDEEEGQRE
TIKLPAGTTSYLVNQDDEED

SEQ ID NO: 133 - protein, 17 aa, synthetic construct
  REGION 1..17: note = EKRHGEWRPSYEKEEDEEEGQRE
HGEWRPSYEKQEDEEEK

SEQ ID NO: 134 - protein, 14 aa, synthetic construct
  REGION 1..14: note = FRAGMENT OF SEQ ID 2
EWRPSYEKEEDEEE

SEQ ID NO: 135 - protein, 14 aa, synthetic construct
  REGION 1..14: note = FRAGMENT OF SEQ ID 2
PSYEKEEDEEEGQR

SEQ ID NO: 136 - protein, 11 aa, synthetic construct
  REGION 1..11: note = FRAGMENT OF SEQ ID 2
EKEEDEEEGQR

SEQ ID NO: 137 - protein, 18 aa, synthetic construct
  REGION 1..18: note = FRAGMENT OF SEQ ID 2
EWRPSYEKEEDEEEGQRE

SEQ ID NO: 138 - protein, 10 aa, synthetic construct
  REGION 1..10: note = FRAGMENT OF SEQ ID 2
KEEDEEEGQR

SEQ ID NO: 139 - protein, 19 aa, synthetic construct
  REGION 1..19: note = FRAGMENT OF SEQ ID 2
VQPGRERWEREEDEEQVDE

SEQ ID NO: 140 - protein, 12 aa, synthetic construct
  REGION 1..12: note = FRAGMENT OF SEQ ID 2
DVVIIPAGHPVA

SEQ ID NO: 141 - protein, 14 aa, synthetic construct
  REGION 1..14: note = FRAGMENT OF SEQ ID 2
HGEWRPSYEKQEDE

SEQ ID NO: 142 - protein, 9 aa, synthetic construct
  REGION 1..9: note = FRAGMENT OF SEQ ID 2
EEDEEEGQR

SEQ ID NO: 143 - protein, 19 aa, synthetic construct
  REGION 1..19: note = FRAGMENT OF SEQ ID 2
HGEWRPSYEKEEDEEEGQR

SEQ ID NO: 144 - protein, 14 aa, synthetic construct
  REGION 1..14: note = FRAGMENT OF SEQ ID 2
EEWRGSQRREDPEE

SEQ ID NO: 145 - protein, 23 aa, synthetic construct
  REGION 1..23: note = FRAGMENT OF SEQ ID 2
REEDEEQVDEEWRGSQRREDPEE

SEQ ID NO: 146 - protein, 9 aa, synthetic construct
  REGION 1..9: note = FRAGMENT OF SEQ ID 2
RHGEWRPSY

SEQ ID NO: 147 - protein, 15 aa, synthetic construct
  REGION 1..15: note = FRAGMENT OF SEQ ID 2
HGEWRPSYEKQEDEE

SEQ ID NO: 148 - protein, 11 aa, synthetic construct
  REGION 1..11: note = FRAGMENT OF SEQ ID 2
VVIIPAGHPVA

SEQ ID NO: 149 - protein, 9 aa, synthetic construct
  REGION 1..9: note = FRAGMENT OF SEQ ID 2
HGEWRPSYE

SEQ ID NO: 150 - protein, 12 aa, synthetic construct
  REGION 1..12: note = FRAGMENT OF SEQ ID 2
KEEDEEEGQRER

SEQ ID NO: 151 - protein, 13 aa, synthetic construct
  REGION 1..13: note = FRAGMENT OF SEQ ID 2
VVIIPAGHPVAIT

SEQ ID NO: 152 - protein, 17 aa, synthetic construct
  REGION 1..17: note = FRAGMENT OF SEQ ID 2
EKRHGEWRPSYEKEEDE

SEQ ID NO: 153 - protein, 17 aa, synthetic construct
  REGION 1..17: note = FRAGMENT OF SEQ ID 2
QVDEEWRGSQRREDPEE

SEQ ID NO: 154 - protein, 24 aa, synthetic construct
  REGION 1..24: note = FRAGMENT OF SEQ ID 2
GDTIKLPAGTTSYLVNQDDEEDLR

SEQ ID NO: 155 - protein, 11 aa, synthetic construct
  REGION 1..11: note = FRAGMENT OF SEQ ID 2
GSEPRVPAQRE

SEQ ID NO: 156 - protein, 15 aa, synthetic construct
  REGION 1..15: note = FRAGMENT OF SEQ ID 2
EEKRHGEWRPSYEKE

SEQ ID NO: 157 - protein, 13 aa, synthetic construct
  REGION 1..13: note = FRAGMENT OF SEQ ID 2
EWRPSYEKEEDEE

SEQ ID NO: 158 - protein, 15 aa, synthetic construct
  REGION 1..15: note = FRAGMENT OF SEQ ID 2
NYDEGSEPRVPAQRE

SEQ ID NO: 159 - protein, 12 aa, synthetic construct
  REGION 1..12: note = FRAGMENT OF SEQ ID 2
VIIPAGHPVAIT

SEQ ID NO: 160 - protein, 11 aa, synthetic construct
  REGION 1..11: note = FRAGMENT OF SEQ ID 2
RHGEWRPSYEK

SEQ ID NO: 161 - protein, 9 aa, synthetic construct
  REGION 1..9: note = FRAGMENT OF SEQ ID 2
NYDEGSEPR

SEQ ID NO: 162 - protein, 12 aa, synthetic construct
  REGION 1..12: note = FRAGMENT OF SEQ ID 2
WRPSYEKEEDEE

SEQ ID NO: 163 - protein, 13 aa, synthetic construct
  REGION 1..13: note = FRAGMENT OF SEQ ID 2
WRPSYEKQEDEEE

SEQ ID NO: 164 - protein, 19 aa, synthetic construct
  REGION 1..19: note = FRAGMENT OF SEQ ID 2
EKRHGEWRPSYEKQEDEEE

SEQ ID NO: 165 - protein, 14 aa, synthetic construct
  REGION 1..14: note = FRAGMENT OF SEQ ID 2
VVIIPAGHPVAITA

SEQ ID NO: 166 - protein, 11 aa, synthetic construct
  REGION 1..11: note = FRAGMENT OF SEQ ID 2
KRHGEWRPSYE

SEQ ID NO: 167 - protein, 16 aa, synthetic construct
  REGION 1..16: note = FRAGMENT OF SEQ ID 2
GSDDNVISQIENPVKE

SEQ ID NO: 168 - protein, 10 aa, synthetic construct
  REGION 1..10: note = FRAGMENT OF SEQ ID 2
VVIIPAGHPV

SEQ ID NO: 169 - protein, 8 aa, synthetic construct
  REGION 1..8: note = FRAGMENT OF SEQ ID 2
HGEWRPSY

SEQ ID NO: 170 - protein, 15 aa, synthetic construct
  REGION 1..15: note = FRAGMENT OF SEQ ID 2
RPSYEKEEDEEEGQR

SEQ ID NO: 171 - protein, 10 aa, synthetic construct
  REGION 1..10: note = FRAGMENT OF SEQ ID 2
HGEWRPSYEK

SEQ ID NO: 172 - protein, 14 aa, synthetic construct
  REGION 1..14: note = FRAGMENT OF SEQ ID 2
KRHGEWRPSYEKEE

SEQ ID NO: 173 - protein, 15 aa, synthetic construct
  REGION 1..15: note = FRAGMENT OF SEQ ID 2
VVIIPAGHPVAITAS

SEQ ID NO: 174 - protein, 23 aa, synthetic construct
  REGION 1..23: note = FRAGMENT OF SEQ ID 2
RGDTIKLPAGTTSYLVNQDDEED

SEQ ID NO: 175 - protein, 18 aa, synthetic construct
  REGION 1..18: note = FRAGMENT OF SEQ ID 2
KRHGEWRPSYEKQEDEEE

SEQ ID NO: 176 - protein, 20 aa, synthetic construct
  REGION 1..20: note = FRAGMENT OF SEQ ID 2
DEEQVDEEWRGSQRREDPEE

SEQ ID NO: 177 - protein, 10 aa, synthetic construct
  REGION 1..10: note = FRAGMENT OF SEQ ID 2
RHGEWRPSYE

SEQ ID NO: 178 - protein, 11 aa, synthetic construct
  REGION 1..11: note = FRAGMENT OF SEQ ID 2
HGEWRPSYEKE

SEQ ID NO: 179 - protein, 18 aa, synthetic construct
  REGION 1..18: note = FRAGMENT OF SEQ ID 2
KRHGEWRPSYEKEEDEEE

SEQ ID NO: 180 - protein, 19 aa, synthetic construct
  REGION 1..19: note = FRAGMENT OF SEQ ID 2
EKRHGEWRPSYEKEEDEEE

SEQ ID NO: 181 - protein, 25 aa, synthetic construct
  REGION 1..25: note = FRAGMENT OF SEQ ID 2
TIKLPAGTTSYLVNQDDEEDLRLVD

SEQ ID NO: 182 - protein, 17 aa, synthetic construct
  REGION 1..17: note = FRAGMENT OF SEQ ID 2
WRPSYEKEEDEEEGQRE

SEQ ID NO: 183 - protein, 17 aa, synthetic construct
  REGION 1..17: note = FRAGMENT OF SEQ ID 2
KRHGEWRPSYEKEEDEE

SEQ ID NO: 184 - protein, 12 aa, synthetic construct
  REGION 1..12: note = FRAGMENT OF SEQ ID 2
VVIIPAGHPVAI

SEQ ID NO: 185 - protein, 13 aa, synthetic construct
  REGION 1..13: note = FRAGMENT OF SEQ ID 2
EWRGSQRREDPEE

SEQ ID NO: 186 - protein, 19 aa, synthetic construct
  REGION 1..19: note = FRAGMENT OF SEQ ID 2
HGEWRPSYEKQEDEEEKQK

SEQ ID NO: 187 - protein, 17 aa, synthetic construct
  REGION 1..17: note = FRAGMENT OF SEQ ID 2
SGSDDNVISQIENPVKE

SEQ ID NO: 188 - protein, 17 aa, synthetic construct
  REGION 1..17: note = FRAGMENT OF SEQ ID 2
RPSYEKEEDEEEGQRER

SEQ ID NO: 189 - protein, 13 aa, synthetic construct
  REGION 1..13: note = FRAGMENT OF SEQ ID 2
EKEEDEEEGQRER

SEQ ID NO: 190 - protein, 11 aa, synthetic construct
  REGION 1..11: note = FRAGMENT OF SEQ ID 2
HGEWRPSYEKQ

SEQ ID NO: 191 - protein, 13 aa, synthetic construct
  REGION 1..13: note = FRAGMENT OF SEQ ID 2
WRPSYEKEEDEEE

SEQ ID NO: 192 - protein, 13 aa, synthetic construct
  REGION 1..13: note = FRAGMENT OF SEQ ID 2
LAKNKNQYLRGFS

SEQ ID NO: 193 - protein, 10 aa, synthetic construct
  REGION 1..10: note = FRAGMENT OF SEQ ID 2
NKNQYLRGFS

SEQ ID NO: 194 - protein, 10 aa, synthetic construct
  REGION 1..10: note = FRAGMENT OF SEQ ID 2
LRGFSKNILE

SEQ ID NO: 195 - protein, 15 aa, synthetic construct
  REGION 1..15: note = FRAGMENT OF SEQ ID 2
LAKNKNQYLRGFSKN

SEQ ID NO: 196 - protein, 11 aa, synthetic construct
  REGION 1..11: note = FRAGMENT OF SEQ ID 2
TVLSPNDRNSY

SEQ ID NO: 197 - protein, 12 aa, synthetic construct
  REGION 1..12: note = FRAGMENT OF SEQ ID 2
QYLRGFSKNILE

SEQ ID NO: 198 - protein, 19 aa, synthetic construct
  REGION 1..19: note = FRAGMENT OF SEQ ID 2
GKAILTVLSPNDRNSYNLE

SEQ ID NO: 199 - protein, 9 aa, synthetic construct
  REGION 1..9: note = FRAGMENT OF SEQ ID 2
RGFSKNILE

SEQ ID NO: 200 - protein, 15 aa, synthetic construct
  REGION 1..15: note = FRAGMENT OF SEQ ID 2
NKNQYLRGFSKNILE

SEQ ID NO: 201 - protein, 15 aa, synthetic construct
  REGION 1..15: note = FRAGMENT OF SEQ ID 2
ASSNLNLLGFGINAE

SEQ ID NO: 202 - protein, 10 aa, synthetic construct
  REGION 1..10: note = FRAGMENT OF SEQ ID 2
ASSNLNLLGF

SEQ ID NO: 203 - protein, 14 aa, synthetic construct
  REGION 1..14: note = FRAGMENT OF SEQ ID 2
LAKNKNQYLRGFSK

SEQ ID NO: 204 - protein, 22 aa, synthetic construct
  REGION 1..22: note = FRAGMENT OF SEQ ID 2
RGDTIKLPAGTTSYLVNQDDEE

SEQ ID NO: 205 - protein, 24 aa, synthetic construct
  REGION 1..24: note = FRAGMENT OF SEQ ID 2
ARLSPGDVVIIPAGHPVAITASSN

SEQ ID NO: 206 - protein, 12 aa, synthetic construct
  REGION 1..12: note = FRAGMENT OF SEQ ID 2
VQRYEARLSPGD

SEQ ID NO: 207 - protein, 20 aa, synthetic construct
  REGION 1..20: note = FRAGMENT OF SEQ ID 2
ARLSPGDVVIIPAGHPVAIT

SEQ ID NO: 208 - protein, 21 aa, synthetic construct
  REGION 1..21: note = FRAGMENT OF SEQ ID 2
RGDTIKLPAGTTSYLVNQDDE

SEQ ID NO: 209 - protein, 18 aa, synthetic construct
  REGION 1..18: note = FRAGMENT OF SEQ ID 2
ARLSPGDVVIIPAGHPVA

SEQ ID NO: 210 - protein, 20 aa, synthetic construct
  REGION 1..20: note = FRAGMENT OF SEQ ID 2
GALMLPHYNSRAIVVLLVNE

SEQ ID NO: 211 - protein, 23 aa, synthetic construct
  REGION 1..23: note = FRAGMENT OF SEQ ID 2
ARLSPGDVVIIPAGHPVAITASS

SEQ ID NO: 212 - protein, 37 aa, synthetic construct
  REGION 1..37: note = FRAGMENT OF SEQ ID 2
LSPGDVVIIPAGHPVAITASSNLNLLGFGINAENNER

SEQ ID NO: 213 - protein, 22 aa, synthetic construct
  REGION 1..22: note = FRAGMENT OF SEQ ID 2
ARLSPGDVVIIPAGHPVAITAS

SEQ ID NO: 214 - protein, 23 aa, synthetic construct
  REGION 1..23: note = FRAGMENT OF SEQ ID 2
LSPGDVVIIPAGHPVAITASSNL

SEQ ID NO: 215 - protein, 21 aa, synthetic construct
  REGION 1..21: note = FRAGMENT OF SEQ ID 2
ARLSPGDVVIIPAGHPVAITA

SEQ ID NO: 216 - protein, 28 aa, synthetic construct
  REGION 1..28: note = FRAGMENT OF SEQ ID 3
NWENVLLGLGVAGSAPGIEGDEIAPLAK

SEQ ID NO: 217 - protein, 17 aa, synthetic construct
  REGION 1..17: note = FRAGMENT OF SEQ ID 3
YDQYKDAWDTSVVAEIK

SEQ ID NO: 218 - protein, 16 aa, synthetic construct
  REGION 1..16: note = FRAGMENT OF SEQ ID 3
SSFDFIDGYDTPVEGR

SEQ ID NO: 219 - protein, 13 aa, synthetic construct
  REGION 1..13: note = FRAGMENT OF SEQ ID 3
GPDTGVDYKDNQM

SEQ ID NO: 220 - protein, 11 aa, synthetic construct
  REGION 1..11: note = FRAGMENT OF SEQ ID 3
ILNLNNNPYFK

SEQ ID NO: 221 - protein, 9 aa, synthetic construct
  REGION 1..9: note = FRAGMENT OF SEQ ID 3
VVGTPAYEE

SEQ ID NO: 222 - protein, 11 aa, synthetic construct
  REGION 1..11: note = FRAGMENT OF SEQ ID 3
IDGYDTPVEGR

SEQ ID NO: 223 - protein, 8 aa, synthetic construct
  REGION 1..8: note = FRAGMENT OF SEQ ID 3
VVGTPAYE

SEQ ID NO: 224 - protein, 11 aa, synthetic construct
  REGION 1..11: note = FRAGMENT OF SEQ ID 3
IYGPDTGVDYK

SEQ ID NO: 225 - protein, 12 aa, synthetic construct
  REGION 1..12: note = FRAGMENT OF SEQ ID 3
VAGSAPGIEGDE

SEQ ID NO: 226 - protein, 16 aa, synthetic construct
  REGION 1..16: note = FRAGMENT OF SEQ ID 3
IYGPDTGVDYKDNQMR

SEQ ID NO: 227 - protein, 12 aa, synthetic construct
  REGION 1..12: note = FRAGMENT OF SEQ ID 3
VVGTPAYEEMVR

SEQ ID NO: 228 - protein, 13 aa, synthetic construct
  REGION 1..13: note = FRAGMENT OF SEQ ID 3
DFIDGYDTPVEGR

SEQ ID NO: 229 - protein, 22 aa, synthetic construct
  REGION 1..22: note = FRAGMENT OF SEQ ID 3
LGLGVAGSAPGIEGDEIAPLAK

SEQ ID NO: 230 - protein, 21 aa, synthetic construct
  REGION 1..21: note = FRAGMENT OF SEQ ID 3
FNAPLAHLIMAGADVLAVPSR

SEQ ID NO: 231 - protein, 16 aa, synthetic construct
  REGION 1..16: note = FRAGMENT OF SEQ ID 3
LGLGVAGSAPGIEGDE

SEQ ID NO: 232 - protein, 20 aa, synthetic construct
  REGION 1..20: note = FRAGMENT OF SEQ ID 3
LGLGVAGSAPGIEGDEIAPL

SEQ ID NO: 233 - protein, 18 aa, synthetic construct
  REGION 1..18: note = FRAGMENT OF SEQ ID 3
VLTVSPYYAEELISGIAR

SEQ ID NO: 234 - protein, 13 aa, synthetic construct
  REGION 1..13: note = FRAGMENT OF SEQ ID 3
EALQAEAGLPVDR

SEQ ID NO: 235 - protein, 15 aa, synthetic construct
  REGION 1..15: note = FRAGMENT OF SEQ ID 3
LGLGVAGSAPGIEGD

SEQ ID NO: 236 - protein, 13 aa, synthetic construct
  REGION 1..13: note = FRAGMENT OF SEQ ID 3
IMAGADVLAVPSR

SEQ ID NO: 237 - protein, 15 aa, synthetic construct
  REGION 1..15: note = FRAGMENT OF SEQ ID 3
GLGVAGSAPGIEGDE

SEQ ID NO: 238 - protein, 14 aa, synthetic construct
  REGION 1..14: note = FRAGMENT OF SEQ ID 3
EALQAEAGLPVDRK

SEQ ID NO: 239 - protein, 21 aa, synthetic construct
  REGION 1..21: note = FRAGMENT OF SEQ ID 3
TGGLGDVLGGLPPAMAANGHR

SEQ ID NO: 240 - protein, 11 aa, synthetic construct
  REGION 1..11: note = FRAGMENT OF SEQ ID 3
LEEQKGPDVMA

SEQ ID NO: 241 - protein, 20 aa, synthetic construct
  REGION 1..20: note = FRAGMENT OF SEQ ID 3
LGVAGSAPGIEGDEIAPLAK

SEQ ID NO: 242 - protein, 21 aa, synthetic construct
  REGION 1..21: note = FRAGMENT OF SEQ ID 3
GLGVAGSAPGIEGDEIAPLAK

SEQ ID NO: 243 - protein, 15 aa, synthetic construct
  REGION 1..15: note = FRAGMENT OF SEQ ID 3
TGGLGDVLGGLPPAM

SEQ ID NO: 244 - protein, 19 aa, synthetic construct
  REGION 1..19: note = FRAGMENT OF SEQ ID 3
NVLLGLGVAGSAPGIEGDE

SEQ ID NO: 245 - protein, 12 aa, synthetic construct
  REGION 1..12: note = FRAGMENT OF SEQ ID 4
TVFDGVLRPGQL

SEQ ID NO: 246 - protein, 16 aa, synthetic construct
  REGION 1..16: note = FRAGMENT OF SEQ ID 4
RLQSQNDQRGEIIHVK

SEQ ID NO: 247 - protein, 15 aa, synthetic construct
  REGION 1..15: note = FRAGMENT OF SEQ ID 5
EGYYGEQQQQPGMTR

SEQ ID NO: 248 - protein, 14 aa, synthetic construct
  REGION 1..14: note = FRAGMENT OF SEQ ID 5
GYYGEQQQQPGMTR

SEQ ID NO: 249 - protein, 16 aa, synthetic construct
  REGION 1..16: note = FRAGMENT OF SEQ ID 5
EEGYYGEQQQQPGMTR

SEQ ID NO: 250 - protein, 20 aa, synthetic construct
  REGION 1..20: note = FRAGMENT OF SEQ ID 5
YYGGEGSSSEQGYYGEGSSE

SEQ ID NO: 251 - protein, 19 aa, synthetic construct
  REGION 1..19: note = FRAGMENT OF SEQ ID 5
YGGEGSSSEQGYYGEGSSE

SEQ ID NO: 252 - protein, 18 aa, synthetic construct
  REGION 1..18: note = FRAGMENT OF SEQ ID 5
SSEEGYYGEQQQQPGMTR

SEQ ID NO: 253 - protein, 17 aa, synthetic construct
  REGION 1..17: note = FRAGMENT OF SEQ ID 5
SEEGYYGEQQQQPGMTR

SEQ ID NO: 254 - protein, 11 aa, synthetic construct
  REGION 1..11: note = FRAGMENT OF SEQ ID 5
QGYYGEGSSEE

SEQ ID NO: 255 - protein, 22 aa, synthetic construct
  REGION 1..22: note = FRAGMENT OF SEQ ID 5
YGGEGSSSEQGYYGEGSSEEGY

SEQ ID NO: 256 - protein, 12 aa, synthetic construct
  REGION 1..12: note = FRAGMENT OF SEQ ID 5
YGEQQQQPGMTR

SEQ ID NO: 257 - protein, 13 aa, synthetic construct
  REGION 1..13: note = FRAGMENT OF SEQ ID 5
YYGEQQQQPGMTR

SEQ ID NO: 258 - protein, 20 aa, synthetic construct
  REGION 1..20: note = FRAGMENT OF SEQ ID 5
SYEESMPMPLEQGWSSSSSE

SEQ ID NO: 259 - protein, 23 aa, synthetic construct
  REGION 1..23: note = FRAGMENT OF SEQ ID 5
YYGEGSSEEGYYGEQQQQPGMTR

SEQ ID NO: 260 - protein, 10 aa, synthetic construct
  REGION 1..10: note = FRAGMENT OF SEQ ID 5
QQQQPGMTRV

SEQ ID NO: 261 - protein, 11 aa, synthetic construct
  REGION 1..11: note = FRAGMENT OF SEQ ID 5
GEQQQQPGMTR

SEQ ID NO: 262 - protein, 21 aa, synthetic construct
  REGION 1..21: note = FRAGMENT OF SEQ ID 5
SYEESMPMPLEQGWSSSSSEY

SEQ ID NO: 263 - protein, 23 aa, synthetic construct
  REGION 1..23: note = FRAGMENT OF SEQ ID 5
YYGGEGSSSEQGYYGEGSSEEGY

SEQ ID NO: 264 - protein, 14 aa, synthetic construct
  REGION 1..14: note = FRAGMENT OF SEQ ID 5
YGEQQQQPGMTRVR

SEQ ID NO: 265 - protein, 21 aa, synthetic construct
  REGION 1..21: note = FRAGMENT OF SEQ ID 5
GEGSSEEGYYGEQQQQPGMTR

SEQ ID NO: 266 - protein, 22 aa, synthetic construct
  REGION 1..22: note = FRAGMENT OF SEQ ID 5
YGEGSSEEGYYGEQQQQPGMTR

SEQ ID NO: 267 - protein, 11 aa, synthetic construct
  REGION 1..11: note = FRAGMENT OF SEQ ID 5
QQQQPGMTRVR

SEQ ID NO: 268 - protein, 25 aa, synthetic construct
  REGION 1..25: note = FRAGMENT OF SEQ ID 5
QYAAQLPSMCRVEPQQCSIFAAGQY

SEQ ID NO: 269 - protein, 12 aa, synthetic construct
  REGION 1..12: note = FRAGMENT OF SEQ ID 6
TVFNGVLRPGQL

SEQ ID NO: 270 - protein, 13 aa, synthetic construct
  REGION 1..13: note = FRAGMENT OF SEQ ID 6
TVFNGVLRPGQLL

SEQ ID NO: 271 - protein, 20 aa, synthetic construct
  REGION 1..20: note = FRAGMENT OF SEQ ID 6
SGFNNELLSEALGVNALVAK

SEQ ID NO: 272 - protein, 9 aa, synthetic construct
  REGION 1..9: note = FRAGMENT OF SEQ ID 6
NGVLRPGQL

SEQ ID NO: 273 - protein, 17 aa, synthetic construct
  REGION 1..17: note = FRAGMENT OF SEQ ID 6
ALVAKRLQGQNDQRGEI

SEQ ID NO: 274 - protein, 10 aa, synthetic construct
  REGION 1..10: note = FRAGMENT OF SEQ ID 6
VPRYSNTPGM

SEQ ID NO: 275 - protein, 10 aa, synthetic construct
  REGION 1..10: note = FRAGMENT OF SEQ ID 6
PRYSNTPGMV

SEQ ID NO: 276 - protein, 9 aa, synthetic construct
  REGION 1..9: note = FRAGMENT OF SEQ ID 6
YSNTPGMVY

SEQ ID NO: 277 - protein, 11 aa, synthetic construct
  REGION 1..11: note = FRAGMENT OF SEQ ID 6
LVPRYSNTPGM

SEQ ID NO: 278 - protein, 10 aa, synthetic construct
  REGION 1..10: note = FRAGMENT OF SEQ ID 6
FYNEGDAPVV

SEQ ID NO: 279 - protein, 12 aa, synthetic construct
  REGION 1..12: note = FRAGMENT OF SEQ ID 6
FYNEGDAPVVAL

SEQ ID NO: 280 - protein, 15 aa, synthetic construct
  REGION 1..15: note = FRAGMENT OF SEQ ID 6
FEPLRRVRSEAGVTE

SEQ ID NO: 281 - protein, 13 aa, synthetic construct
  REGION 1..13: note = FRAGMENT OF SEQ ID 6
FYNEGDAPVVALY

SEQ ID NO: 282 - protein, 11 aa, synthetic construct
  REGION 1..11: note = FRAGMENT OF SEQ ID 6
FYNEGDAPVVA

SEQ ID NO: 283 - protein, 16 aa, synthetic construct
  REGION 1..16: note = FRAGMENT OF SEQ ID 7
HGPVEMPYTLLYPSSK

SEQ ID NO: 284 - protein, 9 aa, synthetic construct
  REGION 1..9: note = FRAGMENT OF SEQ ID 8
LDALEPDNR

SEQ ID NO: 285 - protein, 8 aa, synthetic construct
  REGION 1..8: note = FRAGMENT OF SEQ ID 8
DALEPDNR

SEQ ID NO: 286 - protein, 24 aa, synthetic construct
  REGION 1..24: note = FRAGMENT OF SEQ ID 8
HGSLHKNAMFVPHYNLNANSIIYA

SEQ ID NO: 287 - protein, 20 aa, synthetic construct
  REGION 1..20: note = FRAGMENT OF SEQ ID 8
LAGTSSVINNLPLDVVAATF

SEQ ID NO: 288 - protein, 16 aa, synthetic construct
  REGION 1..16: note = FRAGMENT OF SEQ ID 8
FREGDIIAVPTGIVFW

SEQ ID NO: 289 - protein, 24 aa, synthetic construct
  REGION 1..24: note = FRAGMENT OF SEQ ID 8
GTSSVINNLPLDVVAATFNLQRNE

SEQ ID NO: 290 - protein, 18 aa, synthetic construct
  REGION 1..18: note = FRAGMENT OF SEQ ID 8
KGAIVKVKGGLSIISPPE

SEQ ID NO: 291 - protein, 15 aa, synthetic construct
  REGION 1..15: note = FRAGMENT OF SEQ ID 8
RLAGTSSVINNLPLD

SEQ ID NO: 292 - protein, 25 aa, synthetic construct
  REGION 1..25: note = FRAGMENT OF SEQ ID 8
AGTSSVINNLPLDVVAATFNLQRNE

SEQ ID NO: 293 - protein, 12 aa, synthetic construct
  REGION 1..12: note = FRAGMENT OF SEQ ID 8
AGTSSVINNLPL

SEQ ID NO: 294 - protein, 17 aa, synthetic construct
  REGION 1..17: note = FRAGMENT OF SEQ ID 8
LAGTSSVINNLPLDVVA

SEQ ID NO: 295 - protein, 14 aa, synthetic construct
  REGION 1..14: note = FRAGMENT OF SEQ ID 8
AGTSSVINNLPLDV

SEQ ID NO: 296 - protein, 17 aa, synthetic construct
  REGION 1..17: note = FRAGMENT OF SEQ ID 8
AGRIKTVTSLDLPVLRW

SEQ ID NO: 297 - protein, 16 aa, synthetic construct
  REGION 1..16: note = FRAGMENT OF SEQ ID 8
AGRIKTVTSLDLPVLR

SEQ ID NO: 298 - protein, 15 aa, synthetic construct
  REGION 1..15: note = FRAGMENT OF SEQ ID 8
FREGDIIAVPTGIVF

SEQ ID NO: 299 - protein, 13 aa, synthetic construct
  REGION 1..13: note = FRAGMENT OF SEQ ID 8
AGTSSVINNLPLD

SEQ ID NO: 300 - protein, 13 aa, synthetic construct
  REGION 1..13: note = FRAGMENT OF SEQ ID 8
LAGTSSVINNLPL

SEQ ID NO: 301 - protein, 16 aa, synthetic construct
  REGION 1..16: note = FRAGMENT OF SEQ ID 8
LAGTSSVINNLPLDVV

SEQ ID NO: 302 - protein, 13 aa, synthetic construct
  REGION 1..13: note = FRAGMENT OF SEQ ID 8
EGDIIAVPTGIVF

SEQ ID NO: 303 - protein, 15 aa, synthetic construct
  REGION 1..15: note = FRAGMENT OF SEQ ID 8
LAGTSSVINNLPLDV

SEQ ID NO: 304 - protein, 20 aa, synthetic construct
  REGION 1..20: note = FRAGMENT OF SEQ ID 8
AGRALTVPQNYAVAAKSLSD

SEQ ID NO: 305 - protein, 12 aa, synthetic construct
  REGION 1..12: note = FRAGMENT OF SEQ ID 8
AGRALTVPQNYA

SEQ ID NO: 306 - protein, 14 aa, synthetic construct
  REGION 1..14: note = FRAGMENT OF SEQ ID 8
LAGTSSVINNLPLD

SEQ ID NO: 307 - protein, 23 aa, synthetic construct
  REGION 1..23: note = FRAGMENT OF SEQ ID 8
RAGIARLAGTSSVINNLPLDVVA

SEQ ID NO: 308 - protein, 16 aa, synthetic construct
  REGION 1..16: note = FRAGMENT OF SEQ ID 9
RASSNLNLLGFGINAE

SEQ ID NO: 309 - protein, 12 aa, synthetic construct
  REGION 1..12: note = FRAGMENT OF SEQ ID 9
VTVNEGKGDFEL

SEQ ID NO: 310 - protein, 17 aa, synthetic construct
  REGION 1..17: note = FRAGMENT OF SEQ ID 9
VRASSNLNLLGFGINAE

SEQ ID NO: 311 - protein, 13 aa, synthetic construct
  REGION 1..13: note = FRAGMENT OF SEQ ID 9
VRASSNLNLLGFG

SEQ ID NO: 312 - protein, 17 aa, synthetic construct
  REGION 1..17: note = FRAGMENT OF SEQ ID 9
HPVAVRASSNLNLLGFG

SEQ ID NO: 313 - protein, 16 aa, synthetic construct
  REGION 1..16: note = FRAGMENT OF SEQ ID 9
TKNQVQSYKAKLTPGD

SEQ ID NO: 314 - protein, 15 aa, synthetic construct
  REGION 1..15: note = FRAGMENT OF SEQ ID 9
HPVAVRASSNLNLLG

SEQ ID NO: 315 - protein, 15 aa, synthetic construct
  REGION 1..15: note = FRAGMENT OF SEQ ID 9
KAKLTPGDVFVIPAG

SEQ ID NO: 316 - protein, 19 aa, synthetic construct
  REGION 1..19: note = FRAGMENT OF SEQ ID 9
DLTFPGSAQEVDRLLENQK

SEQ ID NO: 317 - protein, 9 aa, synthetic construct
  REGION 1..9: note = FRAGMENT OF SEQ ID 9
PAGHPVAVR

SEQ ID NO: 318 - protein, 18 aa, synthetic construct
  REGION 1..18: note = FRAGMENT OF SEQ ID 9
AKLTPGDVFVIPAGHPVA

SEQ ID NO: 319 - protein, 21 aa, synthetic construct
  REGION 1..21: note = FRAGMENT OF SEQ ID 9
SYKAKLTPGDVFVIPAGHPVA

SEQ ID NO: 320 - protein, 18 aa, synthetic construct
  REGION 1..18: note = FRAGMENT OF SEQ ID 9
LTPGDVFVIPAGHPVAVR

SEQ ID NO: 321 - protein, 19 aa, synthetic construct
  REGION 1..19: note = FRAGMENT OF SEQ ID 9
VQSYKAKLTPGDVFVIPAG

SEQ ID NO: 322 - protein, 20 aa, synthetic construct
  REGION 1..20: note = FRAGMENT OF SEQ ID 9
YKAKLTPGDVFVIPAGHPVA

SEQ ID NO: 323 - protein, 12 aa, synthetic construct
  REGION 1..12: note = FRAGMENT OF SEQ ID 9
FVIPAGHPVAVR

SEQ ID NO: 324 - protein, 16 aa, synthetic construct
  REGION 1..16: note = FRAGMENT OF SEQ ID 9
YKAKLTPGDVFVIPAG

SEQ ID NO: 325 - protein, 13 aa, synthetic construct
  REGION 1..13: note = FRAGMENT OF SEQ ID 9
DLTFPGSAQEVDR

SEQ ID NO: 326 - protein, 20 aa, synthetic construct
  REGION 1..20: note = FRAGMENT OF SEQ ID 9
AKLTPGDVFVIPAGHPVAVR

SEQ ID NO: 327 - protein, 12 aa, synthetic construct
  REGION 1..12: note = FRAGMENT OF SEQ ID 9
LTPGDVFVIPAG

SEQ ID NO: 328 - protein, 17 aa, synthetic construct
  REGION 1..17: note = FRAGMENT OF SEQ ID 9
SYKAKLTPGDVFVIPAG

SEQ ID NO: 329 - protein, 23 aa, synthetic construct
  REGION 1..23: note = FRAGMENT OF SEQ ID 9
SYKAKLTPGDVFVIPAGHPVAVR

SEQ ID NO: 330 - protein, 11 aa, synthetic construct
  REGION 1..11: note = FRAGMENT OF SEQ ID 9
VIPAGHPVAVR

SEQ ID NO: 331 - protein, 20 aa, synthetic construct
  REGION 1..20: note = FRAGMENT OF SEQ ID 9
QVQSYKAKLTPGDVFVIPAG

SEQ ID NO: 332 - protein, 14 aa, synthetic construct
  REGION 1..14: note = FRAGMENT OF SEQ ID 9
AKLTPGDVFVIPAG

SEQ ID NO: 333 - protein, 21 aa, synthetic construct
  REGION 1..21: note = FRAGMENT OF SEQ ID 9
HPVAVRASSNLNLLGFGINAE

SEQ ID NO: 334 - protein, 22 aa, synthetic construct
  REGION 1..22: note = FRAGMENT OF SEQ ID 9
YKAKLTPGDVFVIPAGHPVAVR

SEQ ID NO: 335 - protein, 23 aa, synthetic construct
  REGION 1..23: note = FRAGMENT OF SEQ ID 9
TKNQVQSYKAKLTPGDVFVIPAG

SEQ ID NO: 336 - protein, 12 aa, synthetic construct
  REGION 1..12: note = FRAGMENT OF SEQ ID 9
PFNLKSSDPIYS

SEQ ID NO: 337 - protein, 8 aa, synthetic construct
  REGION 1..8: note = FRAGMENT OF SEQ ID 9
IEKILLEE

SEQ ID NO: 338 - protein, 16 aa, synthetic construct
  REGION 1..16: note = FRAGMENT OF SEQ ID 9
SRSEPFNLKSSDPIYS

SEQ ID NO: 339 - protein, 13 aa, synthetic construct
  REGION 1..13: note = FRAGMENT OF SEQ ID 9
HPVAVRASSNLNL

SEQ ID NO: 340 - protein, 20 aa, synthetic construct
  REGION 1..20: note = FRAGMENT OF SEQ ID 10
TLFLPQYTDADFILVVLSGK

SEQ ID NO: 341 - protein, 10 aa, synthetic construct
  REGION 1..10: note = FRAGMENT OF SEQ ID 11
EVEERSQNIF

SEQ ID NO: 342 - protein, 12 aa, synthetic construct
  REGION 1..12: note = FRAGMENT OF SEQ ID 11
VEERSQNIFSGF

SEQ ID NO: 343 - protein, 12 aa, synthetic construct
  REGION 1..12: note = FRAGMENT OF SEQ ID 11
ASLQEQEQGQVQ

SEQ ID NO: 344 - protein, 11 aa, synthetic construct
  REGION 1..11: note = FRAGMENT OF SEQ ID 11
QEQEQGQVQSR

SEQ ID NO: 345 - protein, 14 aa, synthetic construct
  REGION 1..14: note = FRAGMENT OF SEQ ID 11
ASLQEQEQGQVQSR

SEQ ID NO: 346 - protein, 13 aa, synthetic construct
  REGION 1..13: note = FRAGMENT OF SEQ ID 11
EVEERSQNIFSGF

SEQ ID NO: 347 - protein, 17 aa, synthetic construct
  REGION 1..17: note = FRAGMENT OF SEQ ID 11
VTDLNNGANQLDPRQRD

SEQ ID NO: 348 - protein, 14 aa, synthetic construct
  REGION 1..14: note = FRAGMENT OF SEQ ID 11
VEHGLSLLQPYASL

SEQ ID NO: 349 - protein, 21 aa, synthetic construct
  REGION 1..21: note = FRAGMENT OF SEQ ID 11
IYVTDLNNGANQLDPRQRDFL

SEQ ID NO: 350 - protein, 19 aa, synthetic construct
  REGION 1..19: note = FRAGMENT OF SEQ ID 11
VTDLNNGANQLDPRQRDFL

SEQ ID NO: 351 - protein, 25 aa, synthetic construct
  REGION 1..25: note = FRAGMENT OF SEQ ID 11
VEHGLSLLQPYASLQEQEQGQVQSR

SEQ ID NO: 352 - protein, 14 aa, synthetic construct
  REGION 1..14: note = FRAGMENT OF SEQ ID 11
VTDLNNGANQLDPR

SEQ ID NO: 353 - protein, 19 aa, synthetic construct
  REGION 1..19: note = FRAGMENT OF SEQ ID 11
IYVTDLNNGANQLDPRQRD

SEQ ID NO: 354 - protein, 20 aa, synthetic construct
  REGION 1..20: note = FRAGMENT OF SEQ ID 11
YVTDLNNGANQLDPRQRDFL

SEQ ID NO: 355 - protein, 15 aa, synthetic construct
  REGION 1..15: note = FRAGMENT OF SEQ ID 11
YVTDLNNGANQLDPR

SEQ ID NO: 356 - protein, 17 aa, synthetic construct
  REGION 1..17: note = FRAGMENT OF SEQ ID 11
STELLSEALGVSSQVAR

SEQ ID NO: 357 - protein, 16 aa, synthetic construct
  REGION 1..16: note = FRAGMENT OF SEQ ID 11
HGLSLLQPYASLQEQE

SEQ ID NO: 358 - protein, 20 aa, synthetic construct
  REGION 1..20: note = FRAGMENT OF SEQ ID 11
SGFSTELLSEALGVSSQVAR

SEQ ID NO: 359 - protein, 13 aa, synthetic construct
  REGION 1..13: note = FRAGMENT OF SEQ ID 12
GAFTPLQYKSYQD

SEQ ID NO: 360 - protein, 15 aa, synthetic construct
  REGION 1..15: note = FRAGMENT OF SEQ ID 12
GLLLPHYTNGASLVY

SEQ ID NO: 361 - protein, 16 aa, synthetic construct
  REGION 1..16: note = FRAGMENT OF SEQ ID 12
FLLAGNKRNPQAYRRE

SEQ ID NO: 362 - protein, 12 aa, synthetic construct
  REGION 1..12: note = FRAGMENT OF SEQ ID 12
ALPTDVLANAYR

SEQ ID NO: 363 - protein, 8 aa, synthetic construct
  REGION 1..8: note = FRAGMENT OF SEQ ID 12
DFLLAGNK

SEQ ID NO: 364 - protein, 8 aa, synthetic construct
  REGION 1..8: note = FRAGMENT OF SEQ ID 12
DVLANAYR

SEQ ID NO: 365 - protein, 9 aa, synthetic construct
  REGION 1..9: note = FRAGMENT OF SEQ ID 12
GAFTPLQYK

SEQ ID NO: 366 - protein, 14 aa, synthetic construct
  REGION 1..14: note = FRAGMENT OF SEQ ID 12
QGDVIALPAGVAHW

SEQ ID NO: 367 - protein, 12 aa, synthetic construct
  REGION 1..12: note = FRAGMENT OF SEQ ID 12
FGAFTPLQYKSY

SEQ ID NO: 368 - protein, 14 aa, synthetic construct
  REGION 1..14: note = FRAGMENT OF SEQ ID 12
FLLAGNKRNPQAYR

SEQ ID NO: 369 - protein, 13 aa, synthetic construct
  REGION 1..13: note = FRAGMENT OF SEQ ID 12
FGAFTPLQYKSYQ

SEQ ID NO: 370 - protein, 15 aa, synthetic construct
  REGION 1..15: note = FRAGMENT OF SEQ ID 12
GLSLLQPYASLQEQE

SEQ ID NO: 371 - protein, 8 aa, synthetic construct
  REGION 1..8: note = FRAGMENT OF SEQ ID 12
AFTPLQYK

SEQ ID NO: 372 - protein, 14 aa, synthetic construct
  REGION 1..14: note = FRAGMENT OF SEQ ID 12
FGAFTPLQYKSYQD

SEQ ID NO: 373 - protein, 13 aa, synthetic construct
  REGION 1..13: note = FRAGMENT OF SEQ ID 12
GDEFGAFTPLQYK

SEQ ID NO: 374 - protein, 15 aa, synthetic construct
  REGION 1..15: note = FRAGMENT OF SEQ ID 12
FGAFTPLQYKSYQDV

SEQ ID NO: 375 - protein, 10 aa, synthetic construct
  REGION 1..10: note = FRAGMENT OF SEQ ID 12
FGAFTPLQYK

SEQ ID NO: 376 - protein, 11 aa, synthetic construct
  REGION 1..11: note = FRAGMENT OF SEQ ID 12
FGAFTPLQYKS

SEQ ID NO: 377 - protein, 14 aa, synthetic construct
  REGION 1..14: note = FRAGMENT OF SEQ ID 12
VYIIQGRGITGPTF

SEQ ID NO: 378 - protein, 13 aa, synthetic construct
  REGION 1..13: note = FRAGMENT OF SEQ ID 12
YIIQGRGITGPTF

SEQ ID NO: 379 - protein, 14 aa, synthetic construct
  REGION 1..14: note = FRAGMENT OF SEQ ID 12
KTNPNSMVSHIAGK

SEQ ID NO: 380 - protein, 13 aa, synthetic construct
  REGION 1..13: note = FRAGMENT OF SEQ ID 12
TNPNSMVSHIAGK

SEQ ID NO: 381 - protein, 12 aa, synthetic construct
  REGION 1..12: note = FRAGMENT OF SEQ ID 12
PNSMVSHIAGKS

SEQ ID NO: 382 - protein, 20 aa, synthetic construct
  REGION 1..20: note = FRAGMENT OF SEQ ID 12
NIDNPNRADTYNPRAGRVTN

SEQ ID NO: 383 - protein, 11 aa, synthetic construct
  REGION 1..11: note = FRAGMENT OF SEQ ID 12
QRDFLLAGNKR

SEQ ID NO: 384 - protein, 12 aa, synthetic construct
  REGION 1..12: note = FRAGMENT OF SEQ ID 12
LLQPYASLQEQE

SEQ ID NO: 385 - protein, 10 aa, synthetic construct
  REGION 1..10: note = FRAGMENT OF SEQ ID 12
QRDFLLAGNK

SEQ ID NO: 386 - protein, 11 aa, synthetic construct
  REGION 1..11: note = FRAGMENT OF SEQ ID 12
QEQEQGQMQSR

SEQ ID NO: 387 - protein, 13 aa, synthetic construct
  REGION 1..13: note = FRAGMENT OF SEQ ID 12
SLLQPYASLQEQE

SEQ ID NO: 388 - protein, 11 aa, synthetic construct
  REGION 1..11: note = FRAGMENT OF SEQ ID 12
ASLQEQEQGQM

SEQ ID NO: 389 - protein, 14 aa, synthetic construct
  REGION 1..14: note = FRAGMENT OF SEQ ID 12
ASLQEQEQGQMQSR

SEQ ID NO: 390 - protein, 9 aa, synthetic construct
  REGION 1..9: note = FRAGMENT OF SEQ ID 12
DFLLAGNKR

SEQ ID NO: 391 - protein, 18 aa, synthetic construct
  REGION 1..18: note = FRAGMENT OF SEQ ID 12
QAFEPIRSVRSQAGTTEF

SEQ ID NO: 392 - protein, 18 aa, synthetic construct
  REGION 1..18: note = FRAGMENT OF SEQ ID 12
KTNPNSMVSHIAGKSSIF

SEQ ID NO: 393 - protein, 21 aa, synthetic construct
  REGION 1..21: note = FRAGMENT OF SEQ ID 12
VRRVIEPRGLLLPHYTNGASL

SEQ ID NO: 394 - protein, 17 aa, synthetic construct
  REGION 1..17: note = FRAGMENT OF SEQ ID 12
FGAFTPLQYKSYQDVYN

SEQ ID NO: 395 - protein, 10 aa, synthetic construct
  REGION 1..10: note = FRAGMENT OF SEQ ID 12
IALPAGVAHW

SEQ ID NO: 396 - protein, 25 aa, synthetic construct
  REGION 1..25: note = FRAGMENT OF SEQ ID 12
RVRQNIDNPNRADTYNPRAGRVTNL

SEQ ID NO: 397 - protein, 21 aa, synthetic construct
  REGION 1..21: note = FRAGMENT OF SEQ ID 12
NIDNPNRADTYNPRAGRVTNL

SEQ ID NO: 398 - protein, 16 aa, synthetic construct
  REGION 1..16: note = FRAGMENT OF SEQ ID 12
GAFTPLQYKSYQDVYN

SEQ ID NO: 399 - protein, 16 aa, synthetic construct
  REGION 1..16: note = FRAGMENT OF SEQ ID 12
PNSMVSHIAGKSSIFR

SEQ ID NO: 400 - protein, 19 aa, synthetic construct
  REGION 1..19: note = FRAGMENT OF SEQ ID 12
RLQAFEPIRSVRSQAGTTE

SEQ ID NO: 401 - protein, 18 aa, synthetic construct
  REGION 1..18: note = FRAGMENT OF SEQ ID 12
TNPNSMVSHIAGKSSIFR

SEQ ID NO: 402 - protein, 11 aa, synthetic construct
  REGION 1..11: note = FRAGMENT OF SEQ ID 13
ELGAPDVGHPM

SEQ ID NO: 403 - protein, 10 aa, synthetic construct
  REGION 1..10: note = FRAGMENT OF SEQ ID 13
LGAPDVGHPM

SEQ ID NO: 404 - protein, 15 aa, synthetic construct
  REGION 1..15: note = FRAGMENT OF SEQ ID 13
ELGAPDVGHPMSEVF

SEQ ID NO: 405 - protein, 12 aa, synthetic construct
  REGION 1..12: note = FRAGMENT OF SEQ ID 13
ELGAPDVGHPMS

SEQ ID NO: 406 - protein, 16 aa, synthetic construct
  REGION 1..16: note = FRAGMENT OF SEQ ID 13
ELGAPDVGHPMSEVFR

SEQ ID NO: 407 - protein, 14 aa, synthetic construct
  REGION 1..14: note = FRAGMENT OF SEQ ID 13
ELGAPDVGHPMSEV

SEQ ID NO: 408 - protein, 13 aa, synthetic construct
  REGION 1..13: note = FRAGMENT OF SEQ ID 13
ELGAPDVGHPMSE

SEQ ID NO: 409 - protein, 12 aa, synthetic construct
  REGION 1..12: note = FRAGMENT OF SEQ ID 13
LGAPDVGHPMSE

SEQ ID NO: 410 - protein, 15 aa, synthetic construct
  REGION 1..15: note = FRAGMENT OF SEQ ID 13
YRELGAPDVGHPMSE

SEQ ID NO: 411 - protein, 13 aa, synthetic construct
  REGION 1..13: note = FRAGMENT OF SEQ ID 13
LGAPDVGHPMSEV

SEQ ID NO: 412 - protein, 14 aa, synthetic construct
  REGION 1..14: note = FRAGMENT OF SEQ ID 13
RELGAPDVGHPMSE

SEQ ID NO: 413 - protein, 16 aa, synthetic construct
  REGION 1..16: note = FRAGMENT OF SEQ ID 14
APTGTFIASGVVVGKD

SEQ ID NO: 414 - protein, 17 aa, synthetic construct
  REGION 1..17: note = FRAGMENT OF SEQ ID 14
LAIVKFSPNEQNKHIGE

SEQ ID NO: 415 - protein, 21 aa, synthetic construct
  REGION 1..21: note = FRAGMENT OF SEQ ID 14
RHQITDTTNGHYAPVTYIQVE

SEQ ID NO: 416 - protein, 19 aa, synthetic construct
  REGION 1..19: note = FRAGMENT OF SEQ ID 14
GDLAIVKFSPNEQNKHIGE

SEQ ID NO: 417 - protein, 18 aa, synthetic construct
  REGION 1..18: note = FRAGMENT OF SEQ ID 14
NPDNPDNPNNPDNPNNPD

SEQ ID NO: 418 - protein, 9 aa, synthetic construct
  REGION 1..9: note = PEPTIDE
QSFILSGNE

SEQ ID NO: 419 - protein, 9 aa, synthetic construct
  REGION 1..9: note = PEPTIDE
ESFLLSGNQ

SEQ ID NO: 420 - protein, 9 aa, synthetic construct
  REGION 1..9: note = PEPTIDE
QSYLLSGNQ

SEQ ID NO: 421 - protein, 9 aa, synthetic construct
  REGION 1..9: note = PEPTIDE
QSFLLSGDQ

SEQ ID NO: 422 - protein, 9 aa, synthetic construct
  REGION 1..9: note = PEPTIDE
QSYLLSGNE

SEQ ID NO: 423 - protein, 9 aa, synthetic construct
  REGION 1..9: note = PEPTIDE
ESFLLSGNE

SEQ ID NO: 424 - protein, 9 aa, synthetic construct
  REGION 1..9: note = PEPTIDE
ESYLLSGNQ

SEQ ID NO: 425 - protein, 9 aa, synthetic construct
  REGION 1..9: note = PEPTIDE
QSFLLSGDE

SEQ ID NO: 426 - protein, 9 aa, synthetic construct
  REGION 1..9: note = PEPTIDE
QSYLLSGDQ

SEQ ID NO: 427 - protein, 9 aa, synthetic construct
  REGION 1..9: note = PEPTIDE
QSFRLSGNQ

SEQ ID NO: 428 - protein, 9 aa, synthetic construct
  REGION 1..9: note = PEPTIDE
QSFLLSYNQ

SEQ ID NO: 429 - protein, 9 aa, synthetic construct
  REGION 1..9: note = PEPTIDE
QFFLLSGNQ

SEQ ID NO: 430 - protein, 9 aa, synthetic construct
  REGION 1..9: note = PEPTIDE
QSFLLSGAQ

SEQ ID NO: 431 - protein, 9 aa, synthetic construct
  REGION 1..9: note = PEPTIDE
QSFLLSGNP

SEQ ID NO: 432 - protein, 9 aa, synthetic construct
  REGION 1..9: note = PEPTIDE
QSFRRSGNQ

SEQ ID NO: 433 - protein, 9 aa, synthetic construct
  REGION 1..9: note = PEPTIDE
QSFLLSYIQ

SEQ ID NO: 434 - protein, 9 aa, synthetic construct
  REGION 1..9: note = PEPTIDE
QFFLLSGNL

SEQ ID NO: 435 - protein, 10 aa, synthetic construct
  REGION 1..10: note = PEPTIDE
QSFLLSGAQA

SEQ ID NO: 436 - protein, 9 aa, synthetic construct
  REGION 1..9: note = PEPTIDE
QSFLLSGNP

SEQ ID NO: 437 - protein, 10 aa, synthetic construct
  REGION 1..10: note = PEPTIDE
QSFLLSGNQQ

SEQ ID NO: 438 - protein, 10 aa, synthetic construct
  REGION 1..10: note = PEPTIDE
QSFLLLSGNQ

SEQ ID NO: 439 - protein, 11 aa, synthetic construct
  REGION 1..11: note = PEPTIDE
AQSFGLLSGNQ

SEQ ID NO: 440 - protein, 11 aa, synthetic construct
  REGION 1..11: note = PEPTIDE
RQSFLLISGNQ

SEQ ID NO: 441 - protein, 10 aa, synthetic construct
  REGION 1..10: note = PEPTIDE
QSFLLSGNQK

SEQ ID NO: 442 - protein, 8 aa, synthetic construct
  REGION 1..8: note = PEPTIDE
QFLLSGNQ

SEQ ID NO: 443 - protein, 8 aa, synthetic construct
  REGION 1..8: note = PEPTIDE
SFLLSGNQ

SEQ ID NO: 444 - protein, 8 aa, synthetic construct
  REGION 1..8: note = PEPTIDE
QSFLLSGN

SEQ ID NO: 445 - protein, 9 aa, synthetic construct
  REGION 1..9: note = PEPTIDE
QSFLLSGNQ

SEQ ID NO: 446 - protein, 8 aa, synthetic construct
  REGION 1..8: note = PEPTIDE
QSFLSGNQ

SEQ ID NO: 447 - protein, 8 aa, synthetic construct
  REGION 1..8: note = PEPTIDE
QSLLSGNQ

SEQ ID NO: 448 - protein, 8 aa, synthetic construct
  REGION 1..8: note = PEPTIDE
SFLLSGNQ

SEQ ID NO: 449 - protein, 8 aa, synthetic construct
  REGION 1..8: note = PEPTIDE
QSFLLSGN

SEQ ID NO: 450 - protein, 7 aa, synthetic construct
  REGION 1..7: note = PEPTIDE
SFLLSGN

SEQ ID NO: 451 - protein, 7 aa, synthetic construct
  REGION 1..7: note = PEPTIDE
QSFSGNQ

SEQ ID NO: 452 - protein, 11 aa, synthetic construct
  REGION 1..11: note = PEPTIDE
HPRPPKPDAPR

SEQ ID NO: 453 - protein, 10 aa, synthetic construct
  REGION 1..10: note = PEPTIDE
LQQAPPPPQR

SEQ ID NO: 454 - protein, 11 aa, synthetic construct
  REGION 1..11: note = PEPTIDE
VGWGEQPWSPY

SEQ ID NO: 455 - protein, 5 aa, synthetic construct
  REGION 1..5: note = PEPTIDE
FHMPP

SEQ ID NO: 456 - protein, 4 aa, synthetic construct
  REGION 1..4: note = PEPTIE
FRRP

SEQ ID NO: 457 - protein, 4 aa, synthetic construct
  REGION 1..4: note = PEPTIDE
FWMA

SEQ ID NO: 458 - protein, 5 aa, synthetic construct
  REGION 1..5: note = PEPTIDE
HMPPS

SEQ ID NO: 459 - protein, 11 aa, synthetic construct
  REGION 1..11: note = PEPTIDE
PVEMPTLLYPS

SEQ ID NO: 460 - protein, 5 aa, synthetic construct
  REGION 1..5: note = PEPTIDE
HMPSS

SEQ ID NO: 461 - protein, 4 aa, synthetic construct
  REGION 1..4: note = PEPTIDE
HRFR

SEQ ID NO: 462 - protein, 4 aa, synthetic construct
  REGION 1..4: note = PEPTIDE
HRRS

SEQ ID NO: 463 - protein, 4 aa, synthetic construct
  REGION 1..4: note = PEPTIDE
HSPR

SEQ ID NO: 464 - protein, 4 aa, synthetic construct
  REGION 1..4: note = PEPTIDE
HWFA

SEQ ID NO: 465 - protein, 4 aa, synthetic construct
  REGION 1..4: note = PEPTIDE
MFRR

SEQ ID NO: 466 - protein, 5 aa, synthetic construct
  REGION 1..5: note = PEPTIDE
MFRRP

SEQ ID NO: 467 - protein, 4 aa, synthetic construct
  REGION 1..4: note = PEPTIDE
MPPS

SEQ ID NO: 468 - protein, 4 aa, synthetic construct
  REGION 1..4: note = PEPTIDE
MPRR

SEQ ID NO: 469 - protein, 4 aa, synthetic construct
  REGION 1..4: note = PEPTIDE
NMPS

SEQ ID NO: 470 - protein, 4 aa, synthetic construct
  REGION 1..4: note = PEPTIDE
PHMP

SEQ ID NO: 471 - protein, 5 aa, synthetic construct
  REGION 1..5: note = PEPTIDE
PHMPS

SEQ ID NO: 472 - protein, 4 aa, synthetic construct
  REGION 1..4: note = PEPTIDE
PRRF

SEQ ID NO: 473 - protein, 4 aa, synthetic construct
  REGION 1..4: note = PEPTIDE
WMKA

SEQ ID NO: 474 - protein, 11 aa, synthetic construct
  REGION 1..11: note = PEPTIDE
DSINALEPDHR

SEQ ID NO: 475 - protein, 9 aa, synthetic construct
  REGION 1..9: note = PEPTIDE
ELTFPGSVQ

SEQ ID NO: 476 - protein, 10 aa, synthetic construct
  REGION 1..10: note = PEPTIDE
ELTFPGSVQE

SEQ ID NO: 477 - protein, 11 aa, synthetic construct
  REGION 1..11: note = PEPTIDE
IFEDAITIPGR

SEQ ID NO: 478 - protein, 13 aa, synthetic construct
  REGION 1..13: note = PEPTIDE
LDALEPDNRIESE

SEQ ID NO: 479 - protein, 10 aa, synthetic construct
  REGION 1..10: note = PEPTIDE
KTLDYWPSLR

SEQ ID NO: 480 - protein, 9 aa, synthetic construct
  REGION 1..9: note = PEPTIDE
RHGEWGPSY

SEQ ID NO: 481 - protein, 11 aa, synthetic construct
  REGION 1..11: note = PEPTIDE
ILVDGSHDIER

SEQ ID NO: 482 - protein, 11 aa, synthetic construct
  REGION 1..11: note = PEPTIDE
ILVDGSHDIER

SEQ ID NO: 483 - protein, 11 aa, synthetic construct
  REGION 1..11: note = PEPTIDE
NLAQAPAQALL

SEQ ID NO: 484 - protein, 7 aa, synthetic construct
  REGION 1..7: note = PEPTIDE
FLPQHTD

SEQ ID NO: 485 - protein, 6 aa, synthetic construct
  REGION 1..6: note = PEPTIDE
LEPDNR

SEQ ID NO: 486 - protein, 6 aa, synthetic construct
  REGION 1..6: note = PEPTIDE
LQSQND

SEQ ID NO: 487 - protein, 11 aa, synthetic construct
  REGION 1..11: note = PEPTIDE
LQSQNDQRGEI

SEQ ID NO: 488 - protein, 14 aa, synthetic construct
  REGION 1..14: note = PEPTIDE
QSQNDQRGEIIHVK

SEQ ID NO: 489 - protein, 8 aa, synthetic construct
  REGION 1..8: note = PEPTIDE
RGEIIHVK

SEQ ID NO: 490 - protein, 8 aa, synthetic construct
  REGION 1..8: note = PEPTIDE
RLQSQNDQ

SEQ ID NO: 491 - protein, 10 aa, synthetic construct
  REGION 1..10: note = PEPTIDE
RLQSQNDQRG

SEQ ID NO: 492 - protein, 14 aa, synthetic construct
  REGION 1..14: note = PEPTIDE
RLQSQNDQRGEIIH

SEQ ID NO: 493 - protein, 9 aa, synthetic construct
  REGION 1..9: note = PEPTIDE
VFDGVLRPG

SEQ ID NO: 494 - protein, 4 aa, synthetic construct
  REGION 1..4: note = PEPTIDE
HNPR

SEQ ID NO: 495 - protein, 4 aa, synthetic construct
  REGION 1..4: note = PEPTIDE
HPMS

SEQ ID NO: 496 - protein, 4 aa, synthetic construct
  REGION 1..4: note = PEPTIDE
HPSF

SEQ ID NO: 497 - protein, 4 aa, synthetic construct
  REGION 1..4: note = PEPTIDE
MPMP

SEQ ID NO: 498 - protein, 4 aa, synthetic construct
  REGION 1..4: note = PEPTIDE
PMPL

SEQ ID NO: 499 - protein, 4 aa, synthetic construct
  REGION 1..4: note = PEPTIDE
PNSM

SEQ ID NO: 500 - protein, 4 aa, synthetic construct
  REGION 1..4: note = PEPTIDE
WDPA

SEQ ID NO: 501 - protein, 6 aa, synthetic construct
  REGION 1..6: note = PEPTIDE
LRGFSK

SEQ ID NO: 502 - protein, 6 aa, synthetic construct
  REGION 1..6: note = PEPTIDE
RSQNIF

SEQ ID NO: 503 - protein, 6 aa, synthetic construct
  REGION 1..6: note = PEPTIDE
YLRGFS

SEQ ID NO: 504 - protein, 9 aa, synthetic construct
  REGION 1..9: note = PEPTIDE
GALMLPHYN

SEQ ID NO: 505 - protein, 11 aa, synthetic construct
  REGION 1..11: note = PEPTIDE
GALMLPHYNSR

SEQ ID NO: 506 - protein, 463 aa, Vicia faba
MAATTLKDSFPLLTLLGIAFLASVCLSSRSDQDNPFVFESNRFQTLFENENGHIRLLQKFDQHSKLLENLQNYRLLEYKSKPHTIFLPQQTDADFILVVLSGKAILTVLLPNDRNSFSLERGDTIKLPAGTIGYLVNRDDEEDLRVLDLVIPVNRPGEPQSFLLSGNQNQPSILSGFSKNILEASFNTDYKEIEKVLLEEHGKEKYHRRGLKDRRQRGQEENVIVKISRKQIEELNKNAKSSSKKSTSSESEPFNLRSREPIYSNKFGKFFEITPKRNPQLQDLNIFVNYVEINEGSLLLPHYNSRAIVIVTVNEGKGDFELVGQRNENQQGLREEYDEEKEQGEEEIRKQVQNYKAKLSPGDVLVIPAGYPVAIKASSNLNLVGFGINAENNQRYFLAGEEDNVISQIHKPVKELAFPGSAQEVDTLLENQKQSHFANAQPRERERGSQEIKDHLYSILGSF

SEQ ID NO: 507 - protein, 446 aa, Cicer arietinum
MAIKARFPLLVLLGIVFLASVCAKSDKENPFFFKSNNCQTLFENENGHVRLLQRFDKRSQLFENLQNYRLMEYNSKPHTLFLPQHNDADFILVVLRGRAILTVLNPNDRNTFKLERGDTIKLPAGTIAYLANRDDNEDLRVLDLAIPVNRPGQFQSFSLSGNENQQSYFQGFSKKILEASFNSDYEEIERVLLEEQEQKPEQRRGHKGRQQSQETDVIVKISREQIEELSKNAKSNCKKSVSSESEPFNLRSRSPIYSNRFGNFFEITPEKNPQLKDLDIFVNSVEIKEGSLLLPHFNSRATVILVVNEGKGEVELVGLRNENEQENKKEDEEEEEDRNVQVQRFQSKLSSGDVVVIPASHPFSINASSDLFLLGFGINAQNNQRNFLAGEEDNVISQIQRPVKEVAFPGSAEEVDRLLKNQRQSHFANAQPQQKRKGSQRIRSPF

SEQ ID NO: 508 - protein, 418 aa, Lens culinaris
SRSDQENPFIFKSNRFQTIYENENGHIRLLQRFDKRSKIFENLQNYRLLEYKSKPHTIFLPQFTDADFILVVLSGKAILTVLNSNDRNSFNLERGDTIKLPAGTIAYLANRDDNEDLRVLDLAIPVNRPGQLQSFLLSGTQNQPSFLSGFSKNILEAAFNTEYEEIEKVLLEEQEQKSQHRRSLRDKRQEITNEDVIVKVSREQIEELSKNAKSSSKKSVSSESEPFNLRSRNPIYSNKFGKFFEITPEKNPQLQDLDIFVNSVEIKEGSLLLPNYNSRAIVIVTVNEGKGDFELVGQRNENQQEQREENDEEEGQEEETTKQVQRYRARLSPGDVLVIPAGHPVAINASSDLNLIGFGINAKNNQRNFLAGEEDNVISQIQRPVKELAFPGSSREVDRLLTNQKQSHFANAQPLQIE

SEQ ID NO: 509 - protein, 526 aa, Pisum elatius
MATTVESRFPLLLFPGIIFLASVCVTYANYDEGSETRVPGQRERGRQEGEKEEKRHGEWRPSYEKEEDEEEKQKYRYQREKEDEEEKQKYRYQREKKEEKEVQPGRERWEREEDEEQVDEEWRGSQRRQDPEERARLRHREERTKRDRRHKREGEEEERSSESQEQRNPFLFKSNKFLTLFENENGHIRRLQRFDKRSDLFENLQNYRLVEYRAKPHTIFLPQHIDADLILVVLNGKAILTVLSPNDRNSYNLERGDTIKIPAGTTSYLVNQDDEEDLRVVDFVIPVNRPGKFEAFGLSENKNQYLRGFSKNILEASLNTKYETIEKVLLEEQEKKPQQLRDRKRRQQGGERDAIIKVSREQIEELRKLAKSSSKKSLPSEFEPFNLRSHKPEYSNKFGKLFEITPEKKYPQLQDLDILVSCVEINKGALMLPHYNSRAIVVLLVNEGKGNLELLGLKNEQQEREDRKERNNEVQRYEARLSPGDVVIIPAGHPVAISASSNLNLLGFGTNAENNQRNFLSGSDDN

SEQ ID NO: 510 - protein, 541 aa, Lathyrus aphaca
MATTIKSRFPLLLLLGIIFLASVCVTWANYDEGSEPRVPGQRERGRQEGEKEEKRHGEWRPSYEEEYDEGLEPKVPGKRERGRQEGEKEEKRHEEWRPSYEKEEDEEEKQKYNYQREKKEHKEVQPGRERWERKQDEKQVEEDEEPGEEQWRGSKRHEDPEERARLRHREEKTKSYVEDNEETSSKEGRNPFLFKSNKFLTLFENENGHIRRLQRFDERSDIFENLQNYRLVEYRAKPHTMFLPQHIDADLILVVLNGKAILTVLSPNDRNSYNLERGDTVKLPAGTTSYLVNQDDEEDLRVVDLAIPVNRPGKFEAFGLSANKNQYLRGFSKNILEASLNTKYETIEKVLLEERRDQKGRQQGQETNAIVKVSREQIEELRKLAKSSSKKSLLSESEPLNLRSQNPKYSNKFGKFFEITPQKKYPQLQDLDVSISCVEINKGALLLPHYNSRSIGILLVNEGKGNLELVGFKNEQQRQRENEETNKKLQRYEARLSSGDVVVIPEGHPVAISASSNLNLLGFGINAANNQRNFLTGSDDN

SEQ ID NO: 511 - protein, 589 aa, Vicia villosa
MATTIKSRFPVLLLLGIIFLTSVCVTYANYDEGREPSVPGQRERGRQEGEKEEKRHGEWRPSEEDEEEKYKYEEGRVPGQRERGRQEGEKEEKRHGKWRPSEEEDEEEKYRYEEGSEPRGPGQRETGRQEGEKEKQRPEREPSYEKEEDEEEKQKYQYHREKKEQREVRPGRERFERHEDEEQWRGIQRHEDPEERARERYRAEIAKRQVEEEREERDIPHEREQRNPFLFKSNKFQTLFQNENGYIRRLQRFDKRSDLFENLQNYRLVEYRAKPHTIFLPQHIDADLIIVVLSGRAILTVLSPDDRNSYNLERGDTIKLPAGTTSYLVNQDDEEDLRVVDLAIPVNRPGKVESFLLSGNKNQYLRGFSKNILEASFNTNYETIERVLLEEQDKESQQSIGQKRRSQRQETNALVKVSREQLEDLKRLAKSSSQEGLSSQFEPINLRSQNPKYSNKFGKVFEITPEKKYPQLQDLDLFVSSVDIKEGALMLPHYNSRAIVVLLVNEGRGNLELVGLKNEQQEQREKEDEQQERNNQVQRYEARLSPGDVVIIPAGHPVAVRASSDLNLLAFGINAENNQRNFLAGSDDN

SEQ ID NO: 512 - protein, 861 aa, Medicago truncatula
MFSGVTGILNRGHKIKGTVVLMRKNVLDINSLTSVGGVIGQGFDILGSTLDNLTAFLGRSVSLQLISATKPDANGKGKLGKATFLEGIITSLPTLGAGQSAFKIHFEWDDDMGIPGAFYIKNFMQTEFFLVSLTLEDIPNHGSIYFVCNSWIYNAKHHKLDRIFFANKAYLPSETPAPLVHYREEELNNLRGDGTGERKEWERIYDYDVYNDLGNPEKGDNHARPVLGGSDTYPYPRRGRTGRKPNPKDPKSESRSDFVYLPRDEAFGHLKSSDFLTYGLKAVSQNVVPALESVIFDLNFTPNEFDSFDEVHGLYEGGIKLPTDVLSKISPLPVLKEIFRTDGEQFLKYPPPKVLQVSRSAWMTDEEFAREMLAGVNPNVICCLQEFPPRSKLDSQVYGDHTSKITKEHLEPNLEGLTVEEAIQNKKLFLLDHHDSIMPYLRRINSTPTKAYATRTILFLSSDKTLKPLAIELSLPHPDGDEHGAVSHVYQPALEGVESTIWLLAKAYVVVNDSCYHQLVSHWLNTHAVVEPFVIATNRHLSYLHPIYKLLYPHYRDTMNINSLARQSLVNDGGIIEKTFLWGRYSMEMSSKVYKNWTLPGQALPADLIKRGMAIEEPSSPCGVKLVVEDYPYAHDGLEIWAAIKTWVQDYVSLYYTTDDILRQDSELQAWWKELVEVGHGDKKNEPWWPKMQAREELVEVCTTVIWIASALHAAVNFGQYSYGGLILNRPTLSRRFMPEKGSAEYNELVKSPQKAYLKTITPKFQTLIDLSVIEILSRHASDEVYLGERDNPNWTSDTRALEAFKKFGNKLAEIEKNLAQRNNDEKLRHRLGPVQMPYTLLHPSSEEGLTFRGIPNSISI

SEQ ID NO: 513 - protein, 857 aa, Glycine soja
MLGGLLHRGHKIKGTVVLMRKNVLDVNSVTSVGGIIGQGLDLVGSTLDTLTAFLGRSVSLQLISATKADANGKGKLGKATFLEGIITSLPTLGAGQSAFKINFEWDDGSGIPGAFYIKNFMQTEFFLVSLTLEDIPNHGSIHFVCNSWIYNAKLFKSDRIFFANQTYLPSETPAPLVKYREEELHNLRGDGTGERKEWERIYDYDVYNDLGDPDKGENHARPVLGGNDTFPYPRRGRTGRKPTRKDPNSESRSNDVYLPRDEAFGHLKSSDFLTYGLKSVSQNVLPLLQSAFDLNFTPREFDSFDEVHGLYSGGIKLPTDIISKISPLPVLKEIFRTDGEQALKFPPPKVIQVSKSAWMTDEEFAREMLAGVNPNLIRCLKDFPPRSKLDSQVYGDHTSQITKEHLEPNLEGLTVDEAIQNKRLFLLDHHDPIMPYLRRINATSTKAYATRTILFLKNDGTLRPLAIELSLPHPQGDQSGAFSQVFLPADEGVESSIWLLAKAYVVVNDSCYHQLVSHWLNTHAVVEPFIIATNRHLSVVHPIYKLLHPHYRDTMNINGLARLSLVNDGGVIEQTFLWGRYSVEMSAVVYKDWVFTDQALPADLIKRGMAIEDPSCPHGIRLVIEDYPYAVDGLEIWDAIKTWVHEYVFLYYKSDDTLREDPELQACWKELVEVGHGDKKNEPWWPKMQTREELVESCAIIIWTASALHAAVNFGQYPYGGLILNRPTLSRRFMPEKGSAEYEELRKNPQKAYLKTITPKFQTLIDLSVIEILSRHASDEVYLGERDNPNWTSDTRALEAFKRFGNKLAQIENKLSERNNDEKLRNRCGPVQMPYTLLLPSSKEGLTFRGIPNSISI

SEQ ID NO: 514 - protein, 860 aa, Phaseolus vulgaris
MFSGVSGLINRGHKLKGTVVLMRKNVLDVNSVTSVGGIVGQGLDILGSTVDNLTAFLGRSVSLQLISATKPDANGKGKLGKATFLEGIITSLPTLGAGQSAFKIHFEWDDEMGIPGAFYIKNFMQTEFYLVSLTLEDIPNHGSLHFLCNSWIYNAKHFKNDRIFFVNQIYLPSETPAPLVKYREEELVNMRGDGTGERKEWDRIYDYDVYNDLGDPDKGENNARPILGGSDTLPYPRRGRTGRRPTRKDPKSESRSSDIYLPRDEAFGHLKSSDFLTYGLKSVSQNFLPALQSAFDLNFTPNEFDSFEEVHGLYSGGIKLPTDVLSKISPLPVLKEIFRTDGEQTLKFPPPKVVQDSKSAWMTDEEFAREMICGVNPNLIRLLQDFPPQSKLDSQVYGDHTSQITKENLEPNLEGLTVDEAIQSKRLFLLDHHDSIMPYLRRINATSSKAYATRTILFLKKDRTLKPLAIELSLPHPGGDKSGVVSQVFLPADEGVESSVWLLAKSYVIVNDSSYHQLVSHWLNTHAVVEPFVIATNRHLSVVHPIYKLLHPHYRDTMNINALARGDLVNHGGIIEKTFVWGRYSMEMSAVIYKDWVFTDQALPADLIKRGIATEDPECPHGLRLFIEDYPYAVDGLEIWDAIKTWVHEYVFLYYKSDDTLKEDPELQAWWKELVEVGHGDKKNEPWWPKMQTREELVEACSIVIWTASALHAAVNFGQYPYGGLILNRPTLSRRFMPEEGSAEYEELKKSPQKALLKTITPKFQTLVDLSVIEILSRHASDEVYLGERDNPNWTSDTRALEAFKRFGKKLSEIEKKLSQRNNDEKLRNRYGPVMMPYTLLFPSSDEGLTFRGIPNSISI

SEQ ID NO: 515 - protein, 498 aa, Vicia sativa
MAKLLALSLSFCFLLFSSCFALREQSQQNECQLERINALEPDNRIESEGGLIETWNPNNRQFRCARVALSRATLQRNALRRPYYSNAPQEIYIQQGNGYFGMVFPGCPETHEEPQQSEQGEGRRYRDSHQKVNRFREGDIIAVPTGIAFWMYNDQDTPVIAISLTDTGSSNNQLDQMPRRFYLAGNQEQEFLRYQHQQGGKQEQDNDGNNIFSGFKRDFLEDAFNVNRHIVDRLQGRNEDEEKGAIVKVKGGLSIIAPPERQARHERGSRQEEDEDEKEERQPSHHKSRRDEDEDDKEKRHSQKGQSRRQGDNGLEETVCTAKLRANIGSSPSPDIYNPQAGRIKTVTSLDLPVLRWLKLSAEHGSLHKNAMFVPHYNLNANSVIYALKGRARLQVVNCNGNTVFDGELEAGRALTVPQNYAVAAKSLSERFTYVAFKTDDRASIARLAGTSSVIDDLPLDVVAATFNMQRNEARQLKSNNPFKFLVPPRQSEMRASA

SEQ ID NO: 516 - protein, 482 aa, Vicia narbonensis
MAKLLALSLSLCFLLFSNSFALREQSQQNECQLERLDALEPDNRIESEGGLIETWNPNNRQFRCAGVALSRVTLQRNALRRPYYSNAPQEIYIQQGNGYFGVVFPGCPETFEEPQESEQRERRRYRDSHQKVNRFREGDIIAVPTGNVLWMYNDQDTPVIAISLTDTGSSNNQLDQIPRRFYLAGNQEQEFLRYQREQGGKQEQENDGNNIFSGFKRDFLEDALNVNRHIVDRLQGRNEDEEKGAIVKVKGGLSIITPPERQRGSRQEEDEDEKEERQPSRRRDESQKGESRRHGDNGLEETVCTAKLRVNIGSSPSPDIYNPQAGRINTVTSLDLPVLRWLKLSAEHGSLRKNALIVPHYNRNANSVIYALKGRARLQVVNCNGNTVFDGELEAGRALTVPQNYAVAAKSLSERFTYVAFKTNDRDGIARLAGTSSVINDLPLDVVAATFNLQRNEARQLKSNNPFKLLVPPRESEKRASA

SEQ ID NO: 517 - protein, 499 aa, Cicer arietinum
  REGION 189..196: note = misc_feature - Xaa can be any naturally occurring amino acid
MAKLLALSLSFCFLLFGSCFALRDQPEQNECQLEHLNALEPDNRIKSEGGLIETWNPSNKQFRCAGVALSRATLQPNSLRRPFYTNAPQEIFIQQGNGYFGMVFPGCVETFEEPRESEQGEGSKFRDSHQKVNRFREGDIIAVPTGVVFWMFNDQDTPVIAVSLIDTSSFQNQLDQMPRRFYLAGNHEXXXXXXXXQQEGSEEEENEGGNIFSGFKRDFLEDALNVNRRIVNKLQGRNEDEEKGAIVKVKGGLSIITPPEKEPRQKRGSRQEEDEDEDEKRQPHRHSRQDEDEDEKRQPRRHSRGGSKSQRDNGFEETICTARLHQNIGSSSSPDIYNPQAGRIKTVTSFDLPALRFLKLSAEFGSLHKNAMFVPHYNLNANSILYALKGRARLQIVNCKGNSVFDGELEAGRALIVPQNFAIAAKSLSDRFSYVAFKTNDRAAIGRLLGASSLINGMPEEVVAAAFNMERNEARQLKFNSPFSFLVPPRSDSDNKAAA

SEQ ID NO: 518 - protein, 576 aa, Lathyrus hirsutus
MAIIIKSRFPLLLLLGIIFLASVCATWANYDEGSEPRVPGQRERGRQEGEKAEKSHEKWRPSYEEEYDEGSEPRVPGKRERGRQEGEKEEKRHGEWRPSHEEEYDEGSEPRVPTHGERGRQEGEKEEKRHEEWRPSYEKEEDEEEKEKYKYQREKKEQKEVQPGREKWERKQDEKHVEEDEDQEEEQWRGSKRREDPEERARLRYREERTKSNVEEETEERRNPFLFKSNKFLTLFENENGHIRRLQRFDERSDIFENLQNYRLVEYKAKPHTMFLPQHIDADLIIVVLNGKAILTVLSPNDRNSYNLERGDTIKLPAGTTSYLVNQDDEEDLRVVDLAIPVNRPGKFEAFGLSANKNQYLRGFSKNILEAFLNTKYETIEKVLLEEQERRDRKGRQQGQETNAIVKVSREQIEELRKLAKSSSKKSLLSESEPINLRSQNPKYSNKFGKLFEITPEKKYPQLQDLDVSISCVEINEGAPLLPHYNSRAIVLLLVNEGKGNLELVGFKNEQQRQRENEERNKKVQRYEARLSPGDVVVIPAGHPVAISASLNLNLVGFGVNAENNQRNFLTGSDDN

SEQ ID NO: 519 - protein, 564 aa, Lathyrus cicera
MATIIKSRFPLLLLLGIIFLASVCVTLANYDEGSEPRVPAQRERGRQEGEKEEKRHGEWRPSHEKEYDEGSEPRVPGRRERGRQEGEKEEKRHGEWRPSYEKEYDEGSEPRVPGRRERGRQEGEKEEKRHGEWRPSYEKEYDEEEKQKYQYEREKEEQKEVQPGRERWERKEDEEKEEDQWRGSQRHEDPEERARLRYRKERTKKYVEEDTEETSSESQGRRNPFLFKSNKFLTLFENENGYIRRLQRFDERSDIFENLQNYRLVEYRAKPHTIFLPQHIDADLILVILNGKAILTVLSPNDRNSYNLERGDTIKLPAGTTSYLVNEDDEEDLRVVDLVIPVNRPGKFEAFDLNQYLGGFSKSVLEASLNTKYETIEKVLLEEQQKQGQETNAIVKVSREQIEELRKLAKSSSKKSLLSELEPVNLRSHSPKYSNKFGKFFEITPEKKYPQLQDLDVSISCVEINEGALLLPHYNSRAIVVVLVNEGKGNLELLGVQNEDEQQERKERNKEVQRYEARLSPGDVVIIPSGHPVAVSASSNLNLLGFGINAENNQRNFLSGSDDN

SEQ ID NO: 520 - protein, 527 aa, Lathyrus sativus
MATIIKSRFPLLLLLGIIFLASVCVTYANYDEGSEPRVPAQRERGRQEGEKEEKRHGEWRPSSEKEYDEGSEPRVPGRRERGRQEGEKEEKRHGEWRPSYEKEYDEEEKQKYQYEREKKEQKEVEPGRERWERKEDEEKEEDQWRGSQRHEDPEERARLRYRKERTKKYVEEDTEETSSESQGRRNPFLFKSNKFLTLFENENGYIRRLQRFDERSDLFENLQNYRLVEYRAKPHTIFLPQHIDADLILVILNGKAILTVLSPNDRNSYNLERGDTIKLPAGTTSYLVNEDDEEDLRVVDLVIPVNRPGKFEAFDLNQYLGGFSKSVLKASLNTKYETIEKVLLEEQQKQGQETNAIVKVSREQIEELRKLAKSSSKKSLLSELEPVNLRSHSPKYSNKFGKFFEITPEKKYPQLQDLDVSISCVEINEGALLLPHYNSRAIVVLLVNEGKGNLELLGVQDEDEQQERKKRNKEVQRYEARLSPSDVVIIPAGHPVAVSASSNLNLLGFGINAENNERNFLSGSDDN

SEQ ID NO: 521 - protein, 463 aa, Medicago truncatula
MAIKAPFQLLMLLGIFFLASVCVSSRDDRHDQENPFFFNANHFQTLFENENGHIRLLQRFDKRSKIFENLQNYRLLEYHSKPHTLFLPQHNDADFILAVLSGKAILTVLNPDNRNSFNLERGDTIKLPAGSIAYLANRDDNEDLRVLDLAIPVNRPGKFQSFSLSGSQNQQSFFSGFSKNILEAAFNANYEEIERVLIEEHEQEPQHRRGLRKDRRQQSQDSNVIVKVSREQIEELSRHAKSSSRRSGSSESAPFNLRSREPIYSNEFGNFFEITPEKNPQLKDLDILVNYAEIREGSLLLPHFNSRATVIVVVDEGKGEFELVGQRNENQQEQREEDEQQEEERSQQVQRYRARLSPGDVYVIPAGHPTVVSASSDLSLLGFGINAENNERNFLAGEEDNVISQIERPVKEVAFPGSAQDVESLLKNQRQSYFANAQPQQREREEGRSQRQRELISSILGVF

SEQ ID NO: 522 - protein, 499 aa, Vicia pannonica
MATTFKSRFSLLLLLGIIFLAFVCVTCANYDEGSEPRVPGQRERGRQEGEKEEQSRERHPQREPSREKEEDEEEKQKYDEGTEPRVPGQRERGRQEGEKEEQRRERHPGQREPSQEEDEEREESDRRQEGSSKSEEQRNPFLFKSNKFLTLFQNGNGHIRLLQRFDKRSDLFENLQNYRLLEYRAKPHTIFLPQHIDADLILVVLSGRAILTVLSPDDRNSYNLERGDTIKLPAGTTSYPLNQDDEEDLRVVDLAISVNRPGKVESFNLSGNKNQYLRGFSENILEASFNTKYETIEKVLLEEQDKESQQPRGQRLQRQETNALVKVSREQVEELKRLARTSSKKGVSSEFEPFNLRSHGPKYSNKFGKFFEITPEKKYPQLQDLDISVSSVEINEGALFLPHYNSRAIVVVLVDEGKGNLELVGFKNEQQEQREKEDEQEERNKQVQRYEAKLSPGDVVIIPAGHPVAVSASSNLNLLGFGINAENNQRNFLTGSDDN

SEQ ID NO: 523 - protein, 515 aa, Vicia ludoviciana
MATTIKLRFPLLLLLGVILLASVCVTCANYDEGSEPRVPGRPEGEKEEKHRGKLRPSYEKEEDEGEKQRYHYEKKEQKEAQPRREKKEQKEEEKQVEEESRESQRYEDPGERARERYRAEIIKRQVEKEREERDRRHQREGEEEEGSSKSRNPFLFKSNNFLTLFENENGHIRLLQRFDKRSDLFENLQNYRLVEYRAKPHTIFLPQHIDADLILVVLSGKAILTVLSPNNRNSYNLKRGDTIKLPAGTTSYLLNSDDEEDLRMVDLAISVNRPGKVESFNLSGNKNQYLRGFSKNILEASFNTKYETIEKVLLEEQDKESQQSIGQKRISQRQETNALVKVSREQIEEPKRLARSSSRKGVSSEFEPINLRSQRPKYSNKFGKFYEISPEKKYPQLQDLDVSVSSVEINEGALLLPHYNSRAIVTVLVNEGKGNLELIGFQNEQQGQREKEDEQQHERNKQVQRYDARLSSGDVVIIPAGHPVAVSASSNLDLLGFGINAENSQRNFLTGSDDN

SEQ ID NO: 524 - protein, 454 aa, Oryza sativa
CRFDRLQAFEPIRSVRSQAGTTEFFDVSNEQFQCTGVSAVRRVIEPRGLLLPHYTNGASLVYIIQGRGITGPTFPGCPESYQQQFQQSGQAQLTESQSQSHKFKDEHQKIHRFRQGDVIALPAGVAHWCYNDGEVPVVAIYVTDLNNGANQLDPRQRDFLLAGNKRNPQAYRREVEERSQNIFSGFSTELLSEALGVSSQVARQLQCQNDQRGEIVRVEHGLSLLQPYASLQEQEQGQVQSRERYQEGQYQQSQYGSGCSNGLDETFCTMKVRQNIDNPNRADTYNPRAGRVTNLNTQNFPILNLVQMSAVKVNLYQNALLSPFWNINAHSVVYITQGRARVQVVNNNGKTVFNGELRRGQLLIIPQHYAVVKKAQREGCAYIAFKTNPNSMVSHIAGKSSIFRALPNDVLANAYRISREEAQRLKHNRGDEFGAFTPIQYKSYQDVYNAAESS

SEQ ID NO: 525 - protein, 500 aa, Zizania latifolia
MNMATINGPTIFFTVCLFLLCHGSLAQLLGQSTSQWQSSHRGSSRQCRFDRLQAFEPVRSVRSQAGTTEFFDASNELFQCAGVSIVRRIIEPRGLLLPQYTNGATIMYIIQGRGITGQTFPGCPESYQQQFQQSMQAQLTGSQSQSQKFKDEHQKINRFRQGDVIALPAGVAHWCYNDGEVPVVAIYVIDINNAANQLDPRQRDFLLAGNMRSPQAYRREVENQSQNIFSGFSAELLSEALGISTGVARQLQCQNDQRGEIVRVEHGLSLLQPYASLQEQEQKQEQPRERYQVTQHQQSQYGGGCSNGLDETFCAMRIWQNIDNPNLADTYNPRAGRVTNLNSQKFPILNLIQMSAVKVNLYQNALLSPFWNINSHSVVYVTQGCARVQVVNNNGKTVFNGELRRGQLLIIPQHYVVVKKAQREGCAYIAFKTNPNSMVSHIVGKSSIFRALPTDVLANAYRISREDAQRLKHNRGDELGAFTPLQYKSYQDVSSVAASS

SEQ ID NO: 526 - protein, 527 aa, Avena sativa
MATTSFPSMLFYFCIFLLFHGSMAQLFGQSSTPWQSSRQGGLRGCRFDRLQAFEPLRQVRSQAGITEYFDEQNEQFRCTGVSVIRRVIEPQGLVLPQYHNAPALVYILQGRGFTGLTFPGCPATFQQQFQPFDQSQFAQGQRQSQTIKDEHQRVQRFKQGDVVALPAGIVHWCYNDGDAPIVAIYVFDVNNNANQLEPRQKEFLLAGNNKREQQSGNNIFSGLSVQLLSEALGISQQAAQRIQSQNDQRGEIIRVSQGLQFLKPIVSQQVPGEQQVYQPIQTQEGQATQYQVGQSTQYQVGKSTPYQGGQSSQYQAGQSWDQSFNGLEENFCSLEARKNIENPQHADTYNPRAGRITRLNSKNFPILNIVQMSATRVNLYQNAILSPFWNINAHSVIYMIQGHARVQVVNNNGQTVFNDILRRGQLLIVPQHFVVLKKAEREGCQYISFKTNPNSMVSHIAGKSSILRALPIDVLANAYRISRQEARNLKNNRGEEFGAFTPKLTQKGFQSYQDIEEGSSSPVRASE

SEQ ID NO: 527 - protein, 495 aa, Oryza sativa
MTISVFSRFSIYFCVLLLCNGSMAQLFDPATNQWQTHRQGSFRECRFERLQAFEPLQNVRSEAGVTEYFDETNELFQCTGTFVIRRVIQPQGLLIPRYANTPGMVYIIQGRGSMGLTFPGCPATYQQQSQQFLFQGESQSQKFIDEHQKIHQFRQGDIVVLPTGVAHWFYNDGDTPVVALYVYDINNSANQLEPRHREFLLAGKNNRVQQVYGRSIQQHSGQNIFNGFSVEPLSEALNINTVTTKRLQSQNDQRGEIIHVKNGLQLLKPTLTQRQEQEQAQYQEVQYSEKPQTSSRWNGLEENLCTIKTRLNIENPSRADSYDPRAGRITSLDSQKFPILNIIQMSATRVNLYQNAILTPFWNVNAHSLMYVIRGRARVQVVSNFGKTVFDGVLRPEQLLIIPQNYVVLKKAQHEGCQYIAINTNANAFVSHLAGVDSVFHALPVDVIANAYCISREEARRLKNNRGDEYGPFPPRLQQQIYPEFSNESKGETSE

SEQ ID NO: 528 - protein, 480 aa, Oryza sativa
LLCHGSMAQIFSLGINPWQNPRQGGSRECRFDRLQAFEPLRKVRHEAGVTEYFDEKNEQFQCTGTLVIRRIIEPQGLLLPRYSNTPGLVYIIQGTGVLGLTFPGCPATYQKQFRHFGLEGGSQRQGKKLRDENQKIHQFRQGDVVALPSGIPHWFYNEGDTPVVALFVFDVNNNANQLEPRQKEFLLAGNNIEQQVSNPSINKHSGQNIFNGFNTKLLSEALGVNIEVTRRLQSQNDRRGDIIRVKNGLRLIKPTITQQQEQTQDQYQQIQYHREQRSTSKYNGLDENFCAIRARLNIENPNHADTYNPRAGRITNLNSQKFSILNLVQMSATRVNLYQNAILSPFWNINAHSLVYTIQGRARVQVVSNHGKAVFNGVLRPGQLLIIPQNYVVMKKAELEGFQFIAFKTNPNAMVNHIAGKNSVLRAMPVDVIANAYRISRQEARSLKNNRGEEIGAFTPRYQQQKIHQEYSNPNESETQ

SEQ ID NO: 529 - protein, 518 aa, Oryza sativa
MATTRFPSLLFYSCIFLLCNGSMAQLFGQSFTPWQSSRQGGLRGCRFDRLQAFEPLRQVRSQAGITEYFDEQNEQFRCAGVSVIRRVIEPQGLLLPQYHNAPGLVYILQGRGFTGLTFPGCPATFQQQFQPFDQARFAQGQSKSQNLKDEHQRVHHIKQGDVVALPAGIVHWCYNDGDAPIVAVYVFDVNNNANQLEPRQKEFLLAGNNKREQQFGQNIFSGFSVQLLSEALGISQQAAQKIQSQNDQRGEIIRVSQGLQFLKPFVSQQGPVEHQAYQPIQSQQEQSTQYQVGQSPQYQEGQSTQYQSGQSWDQSFNGLEENFCSLEARQNIENPKRADTYNPRAGRITHLNSKNFPTLNLVQMSATRVNLYQNAILSPYWNINAHSVMHMIQGRARVQVVNNHGQTVFNDILRRGQLLIIPQHYVVLKKAEREGCQYISFKTTPNSMVSYIAGKTSILRALPVDVLANAYRISRQESQNLKNNRGEEFGAFTPKFAQTGSQSYQDEGESSSTEKASE

SEQ ID NO: 530 - protein, 498 aa, Oryza sativa
MASTNRPIVFFTVCLFLLCDGSLAQQLLGQSTSQWQSSRRGSPRGCRFDRLQAFEPIRSVRSQAGTTEFFDVSNELFQCTGVSVVRRVIEPRGLLLPHYTNGASLVYIIQGRGITGPTFPGCPETYQQQFQQSGQAGLTESQSQSHKFKDEHQKIHRFRQGDVIALPAGVAHWCYNDCEVPVVAIYVTDINNGANQLDPRQRDFLLAGNKRNPQAYRREVEEWSQNIFSGFSTELLSEAFGISNQVARQLQCQNDQKGEIVRVERGLSLLQPYASLQEQEQGQMQSREHYQEGGYQQSQYGSGCPNGLDETFCVNKVRQNIDNPNRADTYNPRAGRVTNLSQNFPILNLVQMSAVKVNLYQNTDTWISMGQEENALLSPFWNINAHSIVYITQGRAQVQVLRRGQLLIVPQHYVVVKKAQREGCAYIAFKTNPNSMVSHIAGKSSIFRALPTDVLANAYRISREEAQRLKHNRGDEFGAFTPLQYKSYQDVYNVAESS

SEQ ID NO: 531 - protein, 491 aa, Oryza brachyantha
MKSSIVFSTICLVLLCHGSLAQLLSQSTSQWQSSRRGSPRQCRFDQLQAFEPIRTVRSQAGVTEFYDVSNELFQCTGVSVVRRVIEPRGLLLPHYSNGATLVYIIQGRGITGPTFPGCPETYQQQFQQSGEAQPFEGQSHKFRDEHQKIHRFRQGDVVALPAGVAHWCYNDGEVPIVAIYVTDIYNSANQLDPRHRDFFLAGNNKVAQQLYRSEARENSKNIFGGFSVELLSEALGISRGVARQLQCQNDQRGEIVRVEHGLALLQPYASVQEQQQEQVQSRDYEQTQYQQKQPQGSCSNGLDETFCTMRLRQNIDNPNLADTYNPKAGRITYLNGQKFPILNLVQMSAVKVNLYQNAVLSPFWNINAHSVVYITQGRARVQVVNNNGKTVFDGELRQGQLLIIPQHHVVLKKAQREGCSYIALKTNPNSIVSHIAGKNSIFRALPGDVVTNAYRISREEAKRIKHNRGDESGVFAPSHAYRSYQDMSVAA

SEQ ID NO: 532 - protein, 492 aa, Brachypodium distachyon
MAHTSFSSFLSYFCLFLLFHGSMAQVLGQVSTWQSSRQGGSRDCSFDRLQAIEPVTQVRSQAGLTEYFDEQNEQFRCAGVFVIRRVIEPRGLLLPRYHNTPGLVYILQGNGFVGLTFPGCPETFREQFQQFRQTQSTLGQSQCQSQKLGDVHQRVHQFTQGDVVALPTGVAHWIYNGGDAPVVIVYVFDVNNNANQLEPRQKEFLLGGNYNGVLQYGQNIFSGFNAQLLSQAFGINEQTSQRIQNQNDGRGDIIRVDNGLQFLKPVVTQQQPEQPFMPIQHQTGQSSRNGLEENFCSLEPRQNIEDPNRADTYNPRAGSITRLNGQNFPILNLVQMSATRVNLQKNAILSPFWNINAHSVVYVIQGHALVQVVNNQGHNVFNGLLHRGQLLIIPQNYVVLKKAESEGYQYIAFKTNANSMVSHIAGKNSILRALPVDVIANAYRISRQEAQNLKNNRGEETGVLTPNFSQSTCQSYQTEDVQSLRPMSHWSE

SEQ ID NO: 533 - protein, 166 aa, Oryza sativa
  SITE 120: note = misc_feature - Xaa can be any naturally occurring amino acid
MASNKVVFSALLLIIVSVLAATATMADHHKDQVVYSLGERCQPGMGYPMYSLPRCRAVVKRQCVGHGAPGGAVDEQLRQDCCRQLAAVDDSWCRCSALNHMVGGIYRELGATDVGHPMAXVFPGCRRGDLERAAASLPAFCNVDIPNGTGGVCYWLGYPRTPRTGH

SEQ ID NO: 534 - protein, 165 aa, Oryza sativa
MASNKVVFSALLLIIVSVLRRDGTMADHHKDQVVYSLGERCQPGMGYPMYSLPRCRAVVKRQCVGHGAPGAVDEQLRQDCCRQLAAVDDSWCRCSALNHMVGGIYRELGATDVGHPMAEVFPGCRRGDLERAAASLPAFCNVDIPNGTGGVCYWLGYPRTPRTGH

SEQ ID NO: 535 - protein, 157 aa, Oryza sativa
MASNKVVISALLVVVVSVLAATTTMADHHQEQVVYTPGQLCQPGIGYPTYPLPRCRAFVKRQCVAPGTVDEQVRRGCCRQLAAIDSSWCRCDALNHMLRIIYRESGAADAGHPMAEVFRGCRRGDIERAAASLPAFCNVDIPNGVGGVCYWLPGTGY

SEQ ID NO: 536 - protein, 605 aa, Oryza rufipogon
MSALTTSQLATSATGFGIADRSAPSSLLRHGFQGLKPRSPAGGDATSLSVTTSARATPKQQRSVQRGSRRFPSVVVYATGAGMNVVFVGAEMAPWSKTGGLGDVLGGLPPAMAANGHRVMVISPRYDQYKDAWDTSVVAEIKVADRYERVRFFHCYKRGVDRVFVDHPSFLEKVWGKTGEKIYGPDTGVDYKDNQMRFSLLCQAPRILNLNNNPYFKGTYGEDVVFVCNDWHTGPLASYLKNNYQPNGIYRNAKVAFCIHNISYQGRFAFEDYPELNLSERFRSSFDFIDGYDTPVEGRKINWMKAGILEADRVLTVSPYYAEELISGIARGCELDNIMRLTGITGIVNGMDVSEWDPSKDKYITAKYDATTAIEAKALNKEALQAEAGLPVDRKIPLIAFIGRLEEQKGPDVMAAAIPELMQEDVQIVLLGTGKKKFEKLLKSMEEKYPGKVRAVVKFNAPLAHLIMAGADVLAVPSRFEPCGLIQLQGMRYGTPCACASTGGLVDTVIEGKTGFHMGRLSVDCKVVEPSDVKKVAATLKRAIKVVGTPAYEEMVRNCMNQDLSWKGPAKNWENVLLGLGVAGSAPGIEGDEIAPLAKENVAAP

SEQ ID NO: 537 - protein, 609 aa, Oryza nivarra
MSALTTSQLATSATGFGIADRSAPSSLLRHGFQGLKPRSPAGGDASSLSVTTSARATPKQQRSVQRGSRRFPSVVVYATGAGMNVVFVGAEMAPWSKTGGLGDVLGGLPPAMAANGHRVMVISPRHDQYKDAWDTSVVAEIKVADRYERVRFFHCYKRGVDRVFIDHPSFLEKVWGKTGEKIYGPDTGVDYKDNQMRFSLLCQAALEAPRILNLNNNPYFKGTYGEDVVFVCNDWHTGPLPSYLKNNYQPNGIYRNAKVAFCIHNISYQGRFAFEDYPELNLSERFRSSFDFIDGYDTPVEGRKINWMKAGILESDRVLTVSPYYAEELISGIARGCELDNIMRLTGITGIVNGMDVSEWDPSKDKYIAAKYDATTAIEAKALNKEALQAEAGLPVDRKIPLIAFIGRLEEQKGPDVMAAAIPELMQENVQIVLLGTGKKKFEKLLKSMEEKYPGKVRAVVKFNAPLAHLIMAGADVLAVPSRFEPCGLIQLQGMRYGTPCACASTGGLVDTVIEGKTGFHMGRLSVDCKVVEPSDVQKVATTLKRAIKIVGTPAYNEMVRNCMNQDLSWKGPAKNWENVLLGLGVAGSAPGVEGEEIAPLAKENVAAP

SEQ ID NO: 538 - protein, 603 aa, Hordeum vulgare
MAALATSQLATSGTVLGVTDRFRRPGFQGLRPRNPADAALGMRTIGASAAPKQSRKAHRGSRRCLSVVVRATGSGMNLVFVGAEMAPWSKTGGLGDVLGGLPPAMAANGHRVMVVSPRYDQYKDAWDTSVISEIKVADEYERVRFFHCYKRGVDRVFIDHPWFLEKVRGKTKEKIYGPDAGTDYEDNQQRFSLLCQAALEAPRILNLNNNPYFSGPYGEDVVFVCNDWHTGLLACYLKSNYQSNGIYRTAKVAFCIHNISYQGRFSFDDFAQLNLPDRFKSSFDFIDGYDKPVEGRKINWMKAGILQADKVLTVSPYYAEELISDEARGCELDNIMRLTGITGIVNGMDVSEWDPTKDKFLAVNYDITTALEAKALNKEALQAEVGLPVDRKVPLVAFIGRLEEQKGPDVMIAAIPEILKEEDVQIILLGTGKKKFEKLLKSMEEKFPGKVRAVVRFNAPLAHQMMAGADLLAVTSRFEPCGLIQLQGMRYGTPCVCASTGGLVDTIVEGKTGFHMGRLSVDCNVVEPADVKKVATTLKRAVKVVGTPAYQEMVKNCMIQDLSWKGPAKNWEDVLLELGVEGSEPGIVGEEIAPLAMENVAAP

SEQ ID NO: 539 - protein, 495 aa, Oryza brachyantha
MATTVFSRFSTYFCVLLLCHGSMAQLFNPSTNPWHNPRQGSSRECRFDRLQPFEPLRKVRSEAGVTEYFDEKNELFQCTGTFVIRRVIQPQGLLVPRYTNAPGLVYIIQGRGSIGLTFPGCPATYQQQFQQFLPQEQSQSQKFRDEHQKIHQFRQGDIVALPAGVAHWFYNDGDAPVVAVYVYDVKNSANQLEPRQREFLLGGNNMRAQQVYGSSAEQHSRQNIFSGFGVEILSEALGISTVTTKRLQSQNDQRGEIIHVKNGLQFLKPTLTQQQEQAQAQYQEVQYSEQQQTSSRWNGLDENFCTIKARMNIENTSRADTYNPRAGRTTSLNSQKFPILNLVQMSATRVNLYQNAILSTFWNVNAHSLVYTIQGRARVQVVSNFGKTVFDGELRPGQLLIIPQHYVVLKKAQREGFRYIAIKTNANAFVSQLVGKNSVFRSLPVDVIANVYRISREQARSLKNNRGEEHGAFAPRSQQQSYPGFSNQSESETSE

SEQ ID NO: 540 - protein, 494 aa, Oryza brachyantha
MATTTFSRFSIYFCVLLLCHGSMAQLFSPTLNPWHSSRRGGSRDCRFDRLQAFEPLRRVRSEAGVTEYFDERNEQFQCTGTFVIRRVIEPQGLLVPRYTNTPGVVYIMQGRGSMGLTFPGCPATYQQQFQQFLPEGQSQSQKFRDEHQKIHQFRQGDIVALPAGVAHWFYNEGDTPVVALYVFDINNSANQLEPRQKDFLLAGNNNREQQVYGRSIEKHSGQNIFSGFNHELLSEALGISTLAAKRLQGQNDHRGEIIRVRNGLQLLKPTFTQQQEQAQSQYQVQYSEKQQESTRCNGLDENFCTINARLNIENPSRADTYNPRAGRITHLNNQKFPILNLVQMSATRVNLYQNAILSPYWNVNAHSLVYMVQGHARVQVVSNLGKTVFNSVLRPGQLLIIPQHYVVLKKAEREGCQYIAFKTNANSIVSQLAGKNSILRAMPVDVVANAYRISREQARDLKNNRGEELGAFTPKFEQQSYPGLSNESESEASE

SEQ ID NO: 541 - protein, 500 aa, Zizania latifolia; identical to SEQ ID NO: 525

SEQ ID NO: 542 - protein, 197 aa, Zea mays
MAKIAAAAAAAAALCFAALVAVAVCQGEVERQRLRDLQCWQEVQESPLDACRQVLDRQLTGGGVGGPFRWGTGLRMRCCQQLQDVSRECRCAAIRSMVRGYEEAMPPLEKGWWPWGRQQQPPPQGGGGGQGGYYYPCSRAGEGYQTQMYPPCRPGTTGPRIGRVRLTKAREYAAGLPMMCRLSEPQECSIFSGGDQY

SEQ ID NO: 543 - protein, 192 aa, Sorghum bicolor
MAKIAAVAATAALCLAALVAVAVGQGVVERQRLKDLQCWQEVQENPLGACRQVLDRQLTGGMRYGIGPFRWGTGLRMRCCQQLQDVSRECRCAAIRSMVRGYEETMPPLEKGWWGQQPQPGYDYPCSQAGEGYGYGESGQQQMYPPCRPGTGQKIARVKLTKARQYAAGMPMMCRLSEPQECSVFSGGDQYY

SEQ ID NO: 544 - protein, 177 aa, Setaria italica
MAKFVVAAATAALCLAALVAMAAGQSGFERQRLRDLRCQREVEENPLWACRQVLDRQLTGGMRYGVGPFRWGTGLRMRCCQQLQDVSRECRCSAVRRMVRGYEEAMPPLEEGPYGYGGEQGEGYYGGGEGGEGYLPFPPRRIGRVRLTKARQYAAGLPMMCRLEPQECSVFSGDQYK

SEQ ID NO: 545 - protein, 336 aa, Staphylococcus aureus
MKGKFLKVSSLFVATLTTATLVSSPAANALSSKAMDNHPQQSQSSKQQTPKIQKGGNLKPLEQREHANVILPNNDRHQITDTTNGHYAPVTYIQVEAPTGTFIASGVVVGKDTLLTNKHVVDATHGDPHALKAFPSAINQDNYPNGGFTAEQITKYSGEGDLAIVKFSPNEQNKHIGEVVKPATMSNNAETQVNQNITVTGYPGDKPVATMWESKGKITYLKGEAMQYDLSTTGGNSGSPVFNEKNEVIGIHWGGVPNEFNGAVFINENVRNFLKQNIEDIHFANDDQPNNPDNPDNPNNPDNPNNPDEPNNPDNPNNPDNPDNGDNNNSDNPDAA

SEQ ID NO: 546 - protein, 11 aa, synthetic construct
  REGION 1..11: note = PEPTIDE
SRAIVIVTVNE

SEQ ID NO: 547 - protein, 8 aa, synthetic construct
  REGION 1..8: note = PEPTIDE
AKLTPGDV

SEQ ID NO: 548 - protein, 10 aa, synthetic construct
  REGION 1..10: note = PEPTIDE
IVIVTVNEGK

SEQ ID NO: 549 - protein, 16 aa, synthetic construct
  REGION 1..16: note = PEPTIDE
LDALEPDNRIESEGGL

SEQ ID NO: 550 - protein, 10 aa, synthetic construct
  REGION 1..10: note = PEPTIDE
RPYYSNAPQE

SEQ ID NO: 551 - protein, 25 aa, synthetic construct
  REGION 1..25: note = PEPTIDE
LDALEPDNRIESEGGLIETWNPNNK

SEQ ID NO: 552 - protein, 11 aa, synthetic construct
  REGION 1..11: note = PEPTIDE
AIVIVTVNEGK

SEQ ID NO: 553 - protein, 16 aa, synthetic construct
  REGION 1..16: note = PEPTIDE
LQVVNCNGNTVFDGEL

SEQ ID NO: 554 - protein, 15 aa, synthetic construct
  REGION 1..15: note = PEPTIDE
QVVNCNGNTVFDGEL

SEQ ID NO: 555 - protein, 10 aa, synthetic construct
  REGION 1..10: note = peptide
IIAVPTGIVF

SEQ ID NO: 556 - protein, 16 aa, synthetic construct
  REGION 1..16: note = PEPTIDE
GRRYRDRHQKVNRFRE

SEQ ID NO: 557 - protein, 11 aa, synthetic construct
  REGION 1..11: note = PEPTIDE
RPYYSNAPQEI

SEQ ID NO: 558 - protein, 12 aa, synthetic construct
  REGION 1..12: note = PEPTIDE
RLDALEPDNRIE

SEQ ID NO: 559 - protein, 14 aa, synthetic construct
  REGION 1..14: note = PEPTIDE
RLDALEPDNRIESE

SEQ ID NO: 560 - protein, 20 aa, synthetic construct
  REGION 1..20: note = PEPTIDE
LDALEPDNRIESEGGLIETW

SEQ ID NO: 561 - protein, 11 aa, synthetic construct
  REGION 1..11: note = PEPTIDE
LDALEPDNRIE

SEQ ID NO: 562 - protein, 18 aa, synthetic construct
  REGION 1..18: note = PEPTIDE
LDALEPDNRIESEGGLIE

SEQ ID NO: 563 - protein, 16 aa, synthetic construct
  REGION 1..16: note = PEPTIDE
LDALEPDNRIESEGGL

SEQ ID NO: 564 - protein, 10 aa, synthetic construct
  REGION 1..10: note = PEPTIDE
RPYYSNAPQE

SEQ ID NO: 565 - protein, 25 aa, synthetic construct
  REGION 1..25: note = PEPTIDE
LDALEPDNRIESEGGLIETWNPNNK

SEQ ID NO: 566 - protein, 27 aa, synthetic construct
  REGION 1..27: note = PEPTIDE
VEHGLSLLQPYASLQEQEQGQVQSRER

SEQ ID NO: 567 - protein, 9 aa, synthetic construct
  REGION 1..9: note = PEPTIDE
RSQNIFSGF

SEQ ID NO: 568 - protein, 14 aa, synthetic construct
  REGION 1..14: note = PEPTIDE
GITGPTFPGCPESY

SEQ ID NO: 569 - protein, 4 aa, synthetic construct
  REGION 1..4: note = PEPTIDE
CNGS

SEQ ID NO: 570 - protein, 5 aa, synthetic construct
  REGION 1..5: note = PEPTIDE
SPREC

SEQ ID NO: 571 - protein, 4 aa, synthetic construct
  REGION 1..4: note = PEPTIDE
PREC

SEQ ID NO: 572 - protein, 5 aa, synthetic construct
  REGION 1..5: note = PEPTIDE
PRECR

SEQ ID NO: 573 - protein, 4 aa, synthetic construct
  REGION 1..4: note = PEPTIDE
CPES

SEQ ID NO: 574 - protein, 4 aa, synthetic construct
  REGION 1..4: note = PEPTIDE
SGCS

SEQ ID NO: 575 - protein, 4 aa, synthetic construct
  REGION 1..4: note = PEPTIDE
CSNG

SEQ ID NO: 576 - protein, 12 aa, synthetic construct
  REGION 1..12: note = PEPTIDE
RSQNIFSGFSTE

SEQ ID NO: 577 - protein, 14 aa, synthetic construct
  REGION 1..14: note = PEPTIDE
VEEWSQNIFSGFST

SEQ ID NO: 578 - protein, 13 aa, synthetic construct
  REGION 1..13: note = PEPTIDE
WSQNIFSGFSTEL

SEQ ID NO: 579 - protein, 12 aa, synthetic construct
  REGION 1..12: note = PEPTIDE
WSQNIFSGFSTE

SEQ ID NO: 580 - protein, 10 aa, synthetic construct
  REGION 1..10: note = PEPTIDE
STSQWQSSRR

SEQ ID NO: 581 - protein, 4 aa, synthetic construct
  REGION 1..4: note = PEPTIDE
NRPI

SEQ ID NO: 582 - protein, 4 aa, synthetic construct
  REGION 1..4: note = PEPTIDE
CDGS

SEQ ID NO: 583 - protein, 4 aa, synthetic construct
  REGION 1..4: note = PEPTIDE
PRGC

SEQ ID NO: 584 - protein, 5 aa, synthetic construct
  REGION 1..5: note = PEPTIDE
PRGCR

SEQ ID NO: 585 - protein, 4 aa, synthetic construct
  REGION 1..4: note = PEPTIDE
RGCR

SEQ ID NO: 586 - protein, 4 aa, synthetic construct
  REGION 1..4: note = PEPTIDE
GCRF

SEQ ID NO: 587 - protein, 4 aa, synthetic construct
  REGION 1..4: note = PEPTIDE
PTFP

SEQ ID NO: 588 - protein, 5 aa, synthetic construct
  REGION 1..5: note = PEPTIDE
PGCPE

SEQ ID NO: 589 - protein, 4 aa, synthetic construct
  REGION 1..4: note = PEPTIDE
GCPE

SEQ ID NO: 590 - protein, 4 aa, synthetic construct
  REGION 1..4: note = PEPTIDE
CPET

SEQ ID NO: 591 - protein, 4 aa, synthetic construct
  REGION 1..4: note = PEPTIDE
AHWC

SEQ ID NO: 592 - protein, 4 aa, synthetic construct
  REGION 1..4: note = PEPTIDE
HWCY

SEQ ID NO: 593 - protein, 4 aa, synthetic construct
  REGION 1..4: note = PEPTIDE
SGCP

SEQ ID NO: 594 - protein, 5 aa, synthetic construct
  REGION 1..5: note = PEPTIDE
SGCPN

SEQ ID NO: 595 - protein, 4 aa, synthetic construct
  REGION 1..4: note = PEPTIDE
GCPN

SEQ ID NO: 596 - protein, 4 aa, synthetic construct
  REGION 1..4: note = PEPTIDE
CPNG

SEQ ID NO: 597 - protein, 5 aa, synthetic construct
  REGION 1..5: note = PEPTIDE
TFCTM

SEQ ID NO: 598 - protein, 4 aa, synthetic construct
  REGION 1..4: note = PEPTIDE
FCTM

SEQ ID NO: 599 - protein, 5 aa, synthetic construct
  REGION 1..5: note = PEPTIDE
FCTMR

SEQ ID NO: 600 - protein, 4 aa, synthetic construct
  REGION 1..4: note = PEPTIDE
CTMR

SEQ ID NO: 601 - protein, 4 aa, synthetic construct
  REGION 1..4: note = PEPTIDE
EGCA

SEQ ID NO: 602 - protein, 13 aa, synthetic construct
  REGION 1..13: note = PEPTIDE
SQNIFSGFSTELL

SEQ ID NO: 603 - protein, 11 aa, synthetic construct
  REGION 1..11: note = PEPTIDE
SQNIFSGFSTE

SEQ ID NO: 604 - protein, 10 aa, synthetic construct
  REGION 1..10: note = PEPTIDE
QNDQRGEIVR

SEQ ID NO: 605 - protein, 12 aa, synthetic construct
  REGION 1..12: note = PEPTIDE
SQNIFSGFSTEL

SEQ ID NO: 606 - protein, 12 aa, synthetic construct
  REGION 1..12: note = PEPTIDE
QLQCQNDQRGEI

SEQ ID NO: 607 - protein, 12 aa, synthetic construct
  REGION 1..12: note = PEPTIDE
LGQSTSQWQSSR

SEQ ID NO: 608 - protein, 15 aa, synthetic construct
  REGION 1..15: note = PEPTIDE
QQLLGQSTSQWQSSR

SEQ ID NO: 609 - protein, 13 aa, synthetic construct
  REGION 1..13: note = PEPTIDE
LLGQSTSQWQSSR

SEQ ID NO: 610 - protein, 9 aa, synthetic construct
  REGION 1..9: note = PEPTIDE
NDQRGEIVR

SEQ ID NO: 611 - protein, 11 aa, synthetic construct
  REGION 1..11: note = PEPTIDE
GQSTSQWQSSR

SEQ ID NO: 612 - protein, 9 aa, synthetic construct
  REGION 1..9: note = PEPTIDE
STSQWQSSR

SEQ ID NO: 613 - protein, 13 aa, synthetic construct
  REGION 1..13: note = PEPTIDE
GITGPTFPGCPET

SEQ ID NO: 614 - protein, 14 aa, synthetic construct
  REGION 1..14: note = PEPTIDE
GITGPTFPGCPETY

SEQ ID NO: 615 - protein, 12 aa, synthetic construct
  REGION 1..12: note = PEPTIDE
SQNIFSGFSTEL

SEQ ID NO: 616 - protein, 12 aa, synthetic construct
  REGION 1..12: note = PEPTIDE
QLQCQNDQRGEI

SEQ ID NO: 617 - protein, 12 aa, synthetic construct
  REGION 1..12: note = PEPTIDE
LGQSTSQWQSSR

SEQ ID NO: 618 - protein, 15 aa, synthetic construct
  REGION 1..15: note = PEPTIDE
QQLLGQSTSQWQSSR

SEQ ID NO: 619 - protein, 13 aa, synthetic construct
  REGION 1..13: note = PEPTIDE
LLGQSTSQWQSSR

SEQ ID NO: 620 - protein, 9 aa, synthetic construct
  REGION 1..9: note = PEPTIDE
IFFANQTYL

SEQ ID NO: 621 - protein, 14 aa, synthetic construct
  REGION 1..14: note = PEPTIDE
EHLEPNLEGLTVEE

SEQ ID NO: 622 - protein, 36 aa, synthetic construct
  REGION 1..36: note = PEPTIDE
IFFANQTYLPSETPAPLVHYREEELNNLRGDGTGER

SEQ ID NO: 623 - protein, 18 aa, synthetic construct
  REGION 1..18: note = PEPTIDE
IHFEWDDDMGIPGAFYIK

SEQ ID NO: 624 - protein, 29 aa, synthetic construct
  REGION 1..29: note = PEPTIDE
IFFANQTYLPSETPAPLVHYREEELNNLR

SEQ ID NO: 625 - protein, 11 aa, synthetic construct
  REGION 1..11: note = PEPTIDE
TEQALPADLIK

SEQ ID NO: 626 - protein, 20 aa, synthetic construct
  REGION 1..20: note = PEPTIDE
EHLEPNLEGLTVEEAIQNKK

SEQ ID NO: 627 - protein, 23 aa, synthetic construct
  REGION 1..23: note = PEPTIDE
ISKEHLEPNLEGLTVEEAIQNKK

SEQ ID NO: 628 - protein, 16 aa, synthetic construct
  REGION 1..16: note = PEPTIDE
LSLPHPQGDEHGAVSY

SEQ ID NO: 629 - protein, 22 aa, synthetic construct
  REGION 1..22: note = PEPTIDE
ISKEHLEPNLEGLTVEEAIQNK

SEQ ID NO: 630 - protein, 19 aa, synthetic construct
  REGION 1..19: note = PEPTIDE
EHLEPNLEGLTVEEAIQNK

SEQ ID NO: 631 - protein, 18 aa, synthetic construct
  REGION 1..18: note = PEPTIDE
LSTTGGNSGSPVFNEKNE

SEQ ID NO: 632 - protein, 17 aa, synthetic construct
  REGION 1..17: note = PEPTIDE
QSFLLSGNQNQQNYLSG

SEQ ID NO: 633 - protein, 16 aa, synthetic construct
  REGION 1..16: note = PEPTIDE
VLDLAIPVNRPGQLQS

SEQ ID NO: 634 - protein, 18 aa, synthetic construct
  REGION 1..18: note = PEPTIDE
VLDLAIPVNRPGQLQSFL

SEQ ID NO: 635 - protein, 15 aa, synthetic construct
  REGION 1..15: note = PEPTIDE
FLLSGNQNQQNYLSG

SEQ ID NO: 636 - protein, 18 aa, synthetic construct
  REGION 1..18: note = PEPTIDE
FLLSGNQNQQNYLSGFSK

SEQ ID NO: 637 - protein, 18 aa, synthetic construct
  REGION 1..18: note = PEPTIDE
DPQNPFIFKSNKFQTLFE

SEQ ID NO: 638 - protein, 19 aa, synthetic construct
  REGION 1..19: note = PEPTIDE
ELAFPGSAQEVDRILENQK

SEQ ID NO: 639 - protein, 11 aa, synthetic construct
  REGION 1..11: note = PEPTIDE
AIVIVTVNEGK

SEQ ID NO: 640 - protein, 18 aa, synthetic construct
  REGION 1..18: note = PEPTIDE
INAVAAKRLQSQNDQRGE

SEQ ID NO: 641 - protein, 14 aa, synthetic construct
  REGION 1..14: note = PEPTIDE
NRAQQQQVYGSSIE

SEQ ID NO: 642 - protein, 10 aa, synthetic construct
  REGION 1..10: note = PEPTIDE
PSTNPWHSPR

SEQ ID NO: 643 - protein, 4 aa, synthetic construct
  REGION 1..4: note = PEPTIDE
CHGS

SEQ ID NO: 644 - protein, 5 aa, synthetic construct
  REGION 1..5: note = PEPTIDE
CHGSM

SEQ ID NO: 645 - protein, 4 aa, synthetic construct
  REGION 1..4: note = PEPTIDE
PWHS

SEQ ID NO: 646 - protein, 4 aa, synthetic construct
  REGION 1..4: note = PEPTIDE
FREC

SEQ ID NO: 647 - protein, 4 aa, synthetic construct
  REGION 1..4: note = PEPTIDE
RECR

SEQ ID NO: 648 - protein, 4 aa, synthetic construct
  REGION 1..4: note = PEPTIDE
ECRF

SEQ ID NO: 649 - protein, 4 aa, synthetic construct
  REGION 1..4: note = PEPTIDE
CRFD

SEQ ID NO: 650 - protein, 5 aa, synthetic construct
  REGION 1..5: note = PEPTIDE
CRFDR

SEQ ID NO: 651 - protein, 4 aa, synthetic construct
  REGION 1..4: note = PEPTIDE
CTGT

SEQ ID NO: 652 - protein, 4 aa, synthetic construct
  REGION 1..4: note = PEPTIDE
FPGC

SEQ ID NO: 653 - protein, 5 aa, synthetic construct
  REGION 1..5: note = PEPTIDE
FPGCP

SEQ ID NO: 654 - protein, 4 aa, synthetic construct
  REGION 1..4: note = PEPTIDE
PGCP

SEQ ID NO: 655 - protein, 5 aa, synthetic construct
  REGION 1..5: note = PEPTIDE
PGCPA

SEQ ID NO: 656 - protein, 6 aa, synthetic construct
  REGION 1..6: note = PEPTIDE
PGCPAT

SEQ ID NO: 657 - protein, 4 aa, synthetic construct
  REGION 1..4: note = PEPTIDE
GCPA

SEQ ID NO: 658 - protein, 4 aa, synthetic construct
  REGION 1..4: note = PEPTIDE
CPAT

SEQ ID NO: 659 - protein, 4 aa, synthetic construct
  REGION 1..4: note = PEPTIDE
ENFC

SEQ ID NO: 660 - protein, 4 aa, synthetic construct
  REGION 1..4: note = PEPTIDE
NFCT

SEQ ID NO: 661 - protein, 5 aa, synthetic construct
  REGION 1..5: note = PEPTIDE
NFCTI

SEQ ID NO: 662 - protein, 4 aa, synthetic construct
  REGION 1..4: note = PEPTIDE
FCTI

SEQ ID NO: 663 - protein, 14 aa, synthetic construct
  REGION 1..14: note = PEPTIDE
AQQQQVYGSSIEQH

SEQ ID NO: 664 - protein, 23 aa, synthetic construct
  REGION 1..23: note = PEPTIDE
AQQQQVYGSSIEQHSGQNIFSGF

SEQ ID NO: 665 - protein, 14 aa, synthetic construct
  REGION 1..14: note = PEPTIDE
AAKRLQSQNDQRGE

SEQ ID NO: 666 - protein, 12 aa, synthetic construct
  REGION 1..12: note = PEPTIDE
QARSLKNNRGEE

SEQ ID NO: 667 - protein, 15 aa, synthetic construct
  REGION 1..15: note = PEPTIDE
FNPSTNPWHSPRQGS

SEQ ID NO: 668 - protein, 12 aa, synthetic construct
  REGION 1..12: note = PEPTIDE
QARSLKNNRGEE

SEQ ID NO: 669 - protein, 26 aa, synthetic construct
  REGION 1..26: note = PEPTIDE
AAASLPAFCNVDIPNGGGGVCYWLAR

SEQ ID NO: 670 - protein, 18 aa, synthetic construct
  REGION 1..18: note = PEPTIDE
VAGSAPGIEGDEIAPLAK

SEQ ID NO: 671 - protein, 22 aa, synthetic construct
  REGION 1..22: note = PEPTIDE
LGVAGSAPGIEGDEIAPLAKEN

SEQ ID NO: 672 - protein, 17 aa, synthetic construct
  REGION 1..17: note = PEPTIDE
GSAPGIEGDEIAPLAKE

SEQ ID NO: 673 - protein, 15 aa, synthetic construct
  REGION 1..15: note = PEPTIDE
VAGSAPGIEGDEIAP

SEQ ID NO: 674 - protein, 19 aa, synthetic construct
  REGION 1..19: note = PEPTIDE
GVAGSAPGIEGDEIAPLAK

SEQ ID NO: 675 - protein, 21 aa, synthetic construct
  REGION 1..21: note = PEPTIDE
GVAGSAPGIEGDEIAPLAKEN

SEQ ID NO: 676 - protein, 20 aa, synthetic construct
  REGION 1..20: note = PEPTIDE
VAGSAPGIEGDEIAPLAKEN

SEQ ID NO: 677 - protein, 15 aa, synthetic construct
  REGION 1..15: note = PEPTIDE
SAPGIEGDEIAPLAK

SEQ ID NO: 678 - protein, 16 aa, synthetic construct
  REGION 1..16: note = PEPTIDE
GSAPGIEGDEIAPLAK

SEQ ID NO: 679 - protein, 17 aa, synthetic construct
  REGION 1..17: note = PEPTIDE
SAPGIEGDEIAPLAKEN

SEQ ID NO: 680 - protein, 15 aa, synthetic construct
  REGION 1..15: note = PEPTIDE
FNPSTNPWHSPRQGS

SEQ ID NO: 681 - protein, 12 aa, synthetic construct
  REGION 1..12: note = PEPTIDE
VDLVIPVNGPGK

SEQ ID NO: 682 - protein, 13 aa, synthetic construct
  REGION 1..13: note = PEPTIDE
LVDLVIPVNGPGK

SEQ ID NO: 683 - protein, 10 aa, synthetic construct
  REGION 1..10: note = PEPTIDE
IKLPAGTTSY

SEQ ID NO: 684 - protein, 11 aa, synthetic construct
  REGION 1..11: note = PEPTIDE
IKLPAGTTSYL

SEQ ID NO: 685 - protein, 12 aa, synthetic construct
  REGION 1..12: note = PEPTIDE
RRNPFLFKSNKF

SEQ ID NO: 686 - protein, 19 aa, synthetic construct
  REGION 1..19: note = PEPTIDE
IENPVKELTFPGSVQEINR

SEQ ID NO: 687 - protein, 14 aa, synthetic construct
  REGION 1..14: note = PEPTIDE
RRNPFLFKSNKFLT

SEQ ID NO: 688 - protein, 14 aa, synthetic construct
  REGION 1..14: note = PEPTIDE
AKPHTIFLPQHIDA

SEQ ID NO: 689 - protein, 15 aa, synthetic construct
  REGION 1..15: note = PEPTIDE
AKPHTIFLPQHIDAD

SEQ ID NO: 690 - protein, 9 aa, synthetic construct
  REGION 1..9: note = PEPTIDE
KQKYRYQRE

SEQ ID NO: 691 - protein, 9 aa, synthetic construct
  REGION 1..9: note = PEPTIDE
KQKYQYQRE

SEQ ID NO: 692 - protein, 4 aa, synthetic construct
  REGION 1..4: note = PEPTIDE
MLPH

SEQ ID NO: 693 - protein, 19 aa, synthetic construct
  REGION 1..19: note = PEPTIDE
RRNPFLFKSNKFLTLFENE

SEQ ID NO: 694 - protein, 14 aa, synthetic construct
  REGION 1..14: note = PEPTIDE
PFLFKSNKFLTLFE

SEQ ID NO: 695 - protein, 20 aa, synthetic construct
  REGION 1..20: note = PEPTIDE
SQERRNPFLFKSNKFLTLFE

SEQ ID NO: 696 - protein, 17 aa, synthetic construct
  REGION 1..17: note = PEPTIDE
RRNPFLFKSNKFLTLFE

SEQ ID NO: 697 - protein, 22 aa, synthetic construct
  REGION 1..22: note = PEPTIDE
SQERRNPFLFKSNKFLTLFENE

SEQ ID NO: 698 - protein, 9 aa, synthetic construct
  REGION 1..9: note = PEPTIDE
LTFPGSVQE

SEQ ID NO: 699 - protein, 13 aa, synthetic construct
  REGION 1..13: note = PEPTIDE
ELTFPGSVQEINR

SEQ ID NO: 700 - protein, 18 aa, synthetic construct
  REGION 1..18: note = PEPTIDE
KNPQLQDLDIFVNYVEIK

SEQ ID NO: 701 - protein, 24 aa, synthetic construct
  REGION 1..24: note = PEPTIDE
PGQLQSFLLSGNQNQQNYLSGFSK

SEQ ID NO: 702 - protein, 14 aa, synthetic construct
  REGION 1..14: note = PEPTIDE
RGPQQYAEWQINEK

SEQ ID NO: 703 - protein, 14 aa, synthetic construct
  REGION 1..14: note = PEPTIDE
VLDLAIPVNRPGQL

SEQ ID NO: 704 - protein, 24 aa, synthetic construct
  REGION 1..24: note = PEPTIDE
GYVGLTFPGCPATHQQQFQLFEQR

SEQ ID NO: 705 - protein, 820 aa, Oryza sativa
MLCLTSSSSSAPAPLLPSLADRPSPGIAGGGGNVRLSVVSSPRRSWPGKVKTNFSVPATARKNKTMVTVVEEVDHLPIYDLDPKLEEFKDHFNYRIKRYLDQKCLIEKHEGGLEEFSKGYLKFGINTVDGATIYREWAPAAQEAQLIGEFNNWNGAKHKMEKDKFGIWSIKISHVNGKPAIPHNSKVKFRFRHGGGAWVDRIPAWIRYATFDASKFGAPYDGVHWDPPACERYVFKHPRPPKPDAPRIYEAHVGMSGEEPEVSTYREFADNVLPRIRANNYNTVQLMAIMEHSYYASFGYHVTNFFAVSSRSGTPEDLKYLVDKAHSLGLRVLMDVVHSHASNNVTDGLNGYDVGQNTHESYFHTGDRGYHKLWDSRLFNYANWEVLRFLLSNLRYWMDEFMFDGFRFDGVTSMLYHHHGINKGFTGNYKEYFSLDTDVDAIVYMMLANHLMHKLLPEATIVAEDVSGMPVLCRPVDEGGVGFDFRLAMAIPDRWIDYLKNKEDRKWSMSEIVQTLTNRRYTEKCIAYAESHDQSIVGDKTIAFLLMDKEMYTGMSDLQPASPTINRGIALQKMIHFITMALGGDGYLNFMGNEFGHPEWIDFPREGNNWSYDKCRRQWSLVDTDHLRYKYMNAFDQAMNALEEEFSFLSSSKQIVSDMNEKDKVIVFERGDLVFVFNFHPNKTYKGYKVGCDLPGKYRVALDSDALVFGGHGRVGHDVDHFTSPEGMPGVPETNFNNRPNSFKVLSPPRTCVAYYRVDEDREELRRGGAVASGKIVTEYIDVEATSGETISGGWKGSEKDDCGKKGMKFVFRSSDEDCK

SEQ ID NO: 706 - protein, 296 aa, Oryza sativa
MDRYQRVERPRPESAIEENEIRITAQGLIRNYVSYATSLLQDRRIKEIVLKAMGQAISKSVAVAEIIKKRVPGLYQDTNISSVSITDVWEPIEEGLVPLEMTRHVSMISITLSPRDLDKNSPGYQTPVYVEQPRQQPRLQQAPPPPQRQVRQPPPDYEDSYVRGRGRGRGRGRGRGWGRGGYGGYGGYGNNQGGYNQGGGYYDNQGGYGGYDNQGGYGGYDNQGGYGGGGYGYNQGRYGNYQENGGYNRGRGGMRGRGNWNYRGGYERGRGGGFPGGRGYGGRGRGRMGGRGGRGN

SEQ ID NO: 707 - protein, 184 aa, Oryza sativa
MALEHLGRRNVAGSLLLLNLLMYVFLLGFAGWALNSSIKNAGADVGVGWGEQPWSPYYRQSAWFASRFHLATFAALAGALGVAAKASAAYHGGRSGASWRPQGLAAAASLGTAAWAATALAFGVACREIHDAAAAGPAGAARGWRMRALEGLTVTLAFTQLLYVLLLHAAVAGERCGLACAADA

SEQ ID NO: 708 - protein, 483 aa, Pisum sativum
MAIKTKLSLTIFLFFLLALLCSNLAVGRKEKDPELTTCKDQCDMQRQYDEEDKRICMERCDDYIKKKQERQKHKEHEEEEEQEQEEDENPYVFEDNDFETKIDTKDGRVLILNKFNEKSKLLKNIENYGLAVLEIKANAFLSPHHYDSEAILFNIKGRGIIGLVAEDRTERFNLEEGDIMRVPAGTPMYLVNRDENEKLYIAAFHMPPSSGSAPVNLEPFFESAGRKPESVLNTFSSKVLQAALKSSKGELETVLDEQKKGRIFKIEKEDVRGLAPKKSLWPFGGPFKSPFNIFSNNPAFSNKFGSLFEVGPSQEKSGLEGLNLMLTLANITKGSMSTIHYNTNANKIALVIDGEGELEMACPHMPSSSSNSRQKKSSISYHNINAKLRPGVMFVVPAGHPFVNIASKKKNLIVVCFEVNAQRNKKLALAGKKNIVSALDKAAKEVAFDIAAEKVDEVFERKEEFFFPYDNEERKEEHGRAVV

SEQ ID NO: 709 - protein, 197 aa, Pisum sativum
MFRRATSTFLSRASATRRFSTDVATPATNSSFVEAWRKVSPNIDPPKTPLEFLKTRPPVPSTIPTKLTVNFVLPYSSQLAAKEVDSVIIPATTGEMGVLPGHVATIAELKPGVLTVQEGTDTTKYFVSSGFRFIHANSVADIIAVEAVPVNQLDRDLVQKGLQEFTQKLNSATTDLEKREAQIGIDVDSALNSALTG

SEQ ID NO: 710 - protein, 156 aa, Oryza sativa
MKIIFFFALLAIAACSASAQFDAVTQVYRQYQLQPHLMLQQQMLSPCGEFVRQQCSTVATPFFQSPVFQLRNCQVMQQQCCQQLRMIAQQSHCQAISSVQAIVQQLRLQQFASVYFDQSQAQAQAMLALNMPSICGIYPSYNTAPCSIPTVGGIWY

SEQ ID NO: 711 - protein, 704 aa, Pisum sativum
MQDSSTMKFSPLDLMTAIIKGKFNPSNDSSQAPASIIFENREFVMILTTSIAVLIGCVVVLIWRRSNSNKSKQIEVPKLVIKKLPELDVDDGKKKVTVFFGTQTGTAEGFAKAIAEEAKARYEKAKFRVVDMDDYAADDDEYLEKLKRETMALFFLATYGDGEPTDNAARFYKWFTEEYEGEEDSFKNLSYGVFGLGNRQYEHFNKVAKVVDDKLLEQGGKRLVPVGLGDDDQCIEDDFTAWKEELWPALDQLLRDEDDTPVATPYTAAVSEYRVVIHDPLDATVDEKKRHNVNGHAVVDAQHPVRANVAVRRELHTPASDRSCTHLEFDISGTGVVYETGDHVGVYCENLSDTVEEAERILGLSPDTYLSIHTDDEEGKPLGGSSLPPPFPPCTLRTALTKYADLLSSPKKSALVALAAHASDPSEADRLRHLASPAGKDEYAEWVISSQRSLLEVMAEFSSAKPPIGVFFAAVAPRLQPRYYSISSSPRMAPSRIHVTCALVHDKMPTGRIHKGVCSTWMKNSVPLEKNQDCSWAPIFVRQSNFRLPADNKVPVIMIGPGTGLAPFRGFLQERLALKEDGAELGPSVLFFGCRNRQVDYIYEDELNHFVNGGALSELIVAFSRDGPTKEYVQHKMMEKASDIWNMISQGAYVYVCGDAKGMARDVHRTLHTILQEQGSLDSSKTESMVKNLQMTGRYLRDVW

SEQ ID NO: 712 - protein, 358 aa, Oryza sativa
MSAYCGKYKDELIKNAAYIGTPGKGILAADESTGTIGKRFASINVENVEENRRSLRELLFTTPGALQHLSGVILFEETLYQKTKDGKPFVDVLKEGGVLPGIKVDKGTVEVAGTNKETTTQGHDDLGKRCAKYYEAGARFAKWRAVLKIGPNEPSQLSIDLNAQGLARYAIICQENGLVPIVEPEILVDGSHDIERCAYVTEKVLAACYKALNEHHVLLEGSLLKPNMVTPGSESKKVSPQLIAEYTVRALQRTVPAAVPAIVFLSGGQSEEEATVNLNAMNKLSTKKPWALSFSFGRALQQSTLKAWGGKTENVVKAQKAFITRCKANSEATLGTYQGDAVLGEGASESLHVKDYKY

SEQ ID NO: 713 - protein, 275 aa, Pisum sativum
MASLQTQMISFYAIFLSILLTTILFFKVNSTETTSFLITKFSPDQQNLIFQGDGYTTKEKLTLTKAVKNTVGRALYSSPIHIWDRETGNVANFVTSFTFVINAPNSYNVADGFTFFIAPVDTKPQTGGGYLGVFNSAEYDKTTQTVAVEFDTFYNAAWDPSNRDRHIGIDVNSIKSVNTKSWKLQNGEEANVVIAFNAATNVLTVSLTYPNSLEEENVTSYTLSDVVSLKDVVPEWVRIGFSATTGAEYAAHEVLSWSFHSELSGTSSSKQAADA

SEQ ID NO: 714 - protein, 484 aa, Oryza sativa
MATTTSLLSSCLCALLLAPLFSQGVDAWESRQGASRQCRFDRLQAFEPLRKVRSEAGDTEYFDERNEQFRCAGVFVIRRVIEPQGLVVPRYSNTPALAYIIQGKGYVGLTFPGCPATHQQQFQLFEQRQSDQAHKFRDEHQKIHEFRQGDVVALPASVAHWFYNGGDTPAVVVYVYDIKSFANQLEPRQKEFLLAGNNQRGQQIFEHSIFQHSGQNIFSGFNTEVLSEALGINTEASKRLQSQNDQRGDIIRVKHGLQLLKPTLTQRQEEHRQYQQVQYREGQYNGLDENFCTIKARVNIENPSRADYYNPRAGRITLLNNQKFPILNLIGMGAARVNLYQNALLSPFWNINAHSVVYIIQGSVRVQVANNQGRSVFNGVLHQGQLLIIPQNHAVIKKAEHNGCQYVAIKTISDPTVSWVAGKNSILRALPVDVIANAYRISRDEARRLKNNRADEIGPFTPRFPQKSQRGYQFLTEGLSLIGM

SEQ ID NO: 715 - protein, 123 aa, Pisum sativum
QKAPRKQLATKAARKSAPATGGVKKPHRFRPGTVALREIRKYQKSTELLIRKLPFQRLVREIAQDFKTDLRFQSSAVSALQEAAEAYLVGLFEDTNLCAIHAKRVTIMPKDIQLARRIRGERA

SEQ ID NO: 716 - protein, 232 aa, Pisum sativum
MAQSVSLSTIASPILSQKPGSSVKSTPPCMASFPLRRQLPRLGLRNVRAQAGGDGDNKDNSVEVHRVNKDDQGTAVERKPRRSSIDISPFGLLDPWSPMRSMRQMLDTMDRIFEDAITIPGRNIGGGEIRVPWEIKDEEHEIRMRFDMPGVSKEDVKVSVEDDVLVIKSDHREENGGEDCWSRKSYSCYDTRLKLPDNCEKEKVKAELKDGVLYITIPKTKIERTVIDVQIQ

SEQ ID NO: 717 - protein, 10 aa, synthetic construct
  REGION 1..10: note = peptide
LDVTPLSLGL

SEQ ID NO: 718 - protein, 12 aa, synthetic construct
  REGION 1..12: note = PEPTIDE
EEGIQLVAEAIR

SEQ ID NO: 719 - protein, 9 aa, synthetic construct
  REGION 1..9: note = PEPTIDE
YSLKPLVPR

SEQ ID NO: 720 - protein, 4 aa, synthetic construct
  REGION 1..4: note = PEPTIDE
WHTA

SEQ ID NO: 721 - protein, 4 aa, synthetic construct
  REGION 1..4: note = PEPTIDE
WHNA

SEQ ID NO: 722 - protein, 4 aa, synthetic construct
  REGION 1..4: note = PEPTIDE
NNPF

SEQ ID NO: 723 - protein, 4 aa, synthetic construct
  REGION 1..4: note = PEPTIDE
MRFR

SEQ ID NO: 724 - protein, 5 aa, synthetic construct
  REGION 1..5: note = PEPTIDE
MPPSS

SEQ ID NO: 725 - protein, 4 aa, synthetic construct
  REGION 1..4: note = PEPTIDE
HMPS

SEQ ID NO: 726 - protein, 5 aa, synthetic construct
  REGION 1..5: note = PEPTIDE
HMPPS

SEQ ID NO: 727 - protein, 4 aa, synthetic construct
  REGION 1..4: note = PEPTIDE
GHPM

SEQ ID NO: 728 - protein, 4 aa, synthetic construct
  REGION 1..4: note = PEPTIDE
FWNA

SEQ ID NO: 729 - protein, 4 aa, synthetic construct
  REGION 1..4: note = PEPTIDE
FHMP

SEQ ID NO: 730 - protein, 11 aa, synthetic construct
  REGION 1..11: note = PEPTIDE
WTIVQGLPIDE

SEQ ID NO: 731 - protein, 9 aa, synthetic construct
  REGION 1..9: note = PEPTIDE
GYPMYPLPR

SEQ ID NO: 732 - protein, 9 aa, synthetic construct
  REGION 1..9: note = PEPTIDE
HGGEGGRPY

SEQ ID NO: 733 - protein, 6 aa, synthetic construct
  REGION 1..6: note = PEPTIDE
LRGFSK

SEQ ID NO: 734 - protein, 9 aa, synthetic construct
  REGION 1..9: note = PEPTIDE
GALMLPHYN

SEQ ID NO: 735 - protein, 11 aa, synthetic construct
  REGION 1..11: note = PEPTIDE
GALMLPHYNSR

SEQ ID NO: 736 - protein, 9 aa, synthetic construct
  REGION 1..9: note = PEPTIDE
VFDGVLRPG

SEQ ID NO: 737 - protein, 6 aa, synthetic construct
  REGION 1..6: note = PEPTIDE
LQSQND

SEQ ID NO: 738 - protein, 11 aa, synthetic construct
  REGION 1..11: note = PEPTIDE
LQSQNDQRGEI

SEQ ID NO: 739 - protein, 14 aa, synthetic construct
  REGION 1..14: note = PEPTIDE
QSQNDQRGEIIHVK

SEQ ID NO: 740 - protein, 8 aa, synthetic construct
  REGION 1..8: note = PEPTIDE
RGEIIHVK

SEQ ID NO: 741 - protein, 8 aa, synthetic construct
  REGION 1..8: note = PEPTIDE
RLQSQNDQ

SEQ ID NO: 742 - protein, 10 aa, synthetic construct
  REGION 1..10: note = PEPTIDE
RLQSQNDQRG

SEQ ID NO: 743 - protein, 14 aa, synthetic construct
  REGION 1..14: note = PEPTIDE
RLQSQNDQRGEIIH

SEQ ID NO: 744 - protein, 4 aa, synthetic construct
  REGION 1..4: note = PEPTIDE
MPMP

SEQ ID NO: 745 - protein, 4 aa, synthetic construct
  REGION 1..4: note = PEPTIDE
PMPL

SEQ ID NO: 746 - protein, 6 aa, synthetic construct
  REGION 1..6: note = PEPTIDE
LEPDNR

SEQ ID NO: 747 - protein, 13 aa, synthetic construct
  REGION 1..13: note = PEPTIDE
GIARLAGTSSVIN

SEQ ID NO: 748 - protein, 6 aa, synthetic construct
  REGION 1..6: note = PEPTIDE
RSQNIF

SEQ ID NO: 749 - protein, 4 aa, synthetic construct
  REGION 1..4: note = PEPTIDE
PNSM

SEQ ID NO: 750 - protein, 4 aa, synthetic construct
  REGION 1..4: note = PEPTIDE
GHPM

SEQ ID NO: 751 - protein, 4 aa, synthetic construct
  REGION 1..4: note = PEPTIDE
HPMS

SEQ ID NO: 752 - protein, 7 aa, synthetic construct
  REGION 1..7: note = PEPTIDE
FLPQHTD

SEQ ID NO: 753 - protein, 7 aa, synthetic construct
  REGION 1..7: note = PEPTIDE
EWQINEK

SEQ ID NO: 754 - protein, 13 aa, synthetic construct
  REGION 1..13: note = PEPTIDE
GPQQYAEWQINEK

SEQ ID NO: 755 - protein, 8 aa, synthetic construct
  REGION 1..8: note = PEPTIDE
PQQYAEWQ

SEQ ID NO: 756 - protein, 7 aa, synthetic construct
  REGION 1..7: note = PEPTIDE
RGPQQYA

SEQ ID NO: 757 - protein, 4 aa, synthetic construct
  REGION 1..4: note = PEPTIDE
HNPR

SEQ ID NO: 758 - protein, 4 aa, synthetic construct
  REGION 1..4: note = PEPTIDE
WHNR

SEQ ID NO: 759 - protein, 4 aa, synthetic construct
  REGION 1..4: note = PEPTIDE
WDPA

SEQ ID NO: 760 - protein, 4 aa, synthetic construct
  REGION 1..4: note = PEPTIDE
HPSF

SEQ ID NO: 761 - protein, 22 aa, synthetic construct
  REGION 1..22: note = PEPTIDE
PGQLQSFLLSGNQNQQNYLSGF

SEQ ID NO: 762 - protein, 22 aa, synthetic construct
  REGION 1..22: note = PEPTIDE
QLQSFLLSGNQNQQNYLSGFSK

SEQ ID NO: 763 - protein, 12 aa, synthetic construct
  REGION 1..12: note = PEPTIDE
QSFLLSGNQNQQ

SEQ ID NO: 764 - protein, 12 aa, synthetic construct
  REGION 1..12: note = PEPTIDE
PGQLQSFLLSGN

SEQ ID NO: 765 - protein, 9 aa, synthetic construct
  REGION 1..9: note = PEPTIDE
QSFLLSGNQ

SEQ ID NO: 766 - protein, 12 aa, synthetic construct
  REGION 1..12: note = PEPTIDE
QNQQNYLSGFSK

SEQ ID NO: 767 - protein, 6 aa, synthetic construct
  REGION 1..6: note = PEPTIDE
YLRGFS

SEQ ID NO: 768 - protein, 11 aa, synthetic construct
  REGION 1..11: note = PEPTIDE
PVEMPTLLYPS

SEQ ID NO: 769 - protein, 13 aa, synthetic construct
  REGION 1..13: note = PEPTIDE
RGPQQYAEWQINE

SEQ ID NO: 770 - protein, 24 aa, synthetic construct
  REGION 1..24: note = PEPTIDE
GYVGLTFPGCPATHQQQFQLFEQR

SEQ ID NO: 771 - protein, 18 aa, synthetic construct
  REGION 1..18: note = PEPTIDE
KNPQLQDLDIFVNYVEIK

SEQ ID NO: 772 - protein, 24 aa, synthetic construct
  REGION 1..24: note = PEPTIDE
PGQLQSFLLSGNQNQQNYLSGFSK

SEQ ID NO: 773 - protein, 14 aa, synthetic construct
  REGION 1..14: note = PEPTIDE
RGPQQYAEWQINEK

SEQ ID NO: 774 - protein, 14 aa, synthetic construct
  REGION 1..14: note = PEPTIDE
VLDLAIPVNRPGQL

SEQ ID NO: 775 - protein, 14 aa, synthetic construct
  REGION 1..14: note = PEPTIDE
RGPQQYAEWQINEK